European Patent Specification EP 3 684 423 B1, published March 29, 2023. Title: Adeno-Associated Virus Variant Capsids and Methods of Use Thereof. Applicant: 4D Molecular Therapeutics Inc. The sequence listing filed with the application follows.

SEQUENCE LISTING (69 sequences)

SEQ ID NO: 1 - protein, 736 aa, Adeno-associated virus 1
MAADGYLPDWLEDNLSEGIREWWDLKPGAPKPKANQQKQDDGRGLVLPGYKYLGPFNGLDKGEPVNAADAAALEHDKAYDQQLKAGDNPYLRYNHADAEFQERLQEDTSFGGNLGRAVFQAKKRVLEPLGLVEEGAKTAPGKKRPVEQSPQEPDSSSGIGKTGQQPAKKRLNFGQTGDSESVPDPQPLGEPPATPAAVGPTTMASGGGAPMADNNEGADGVGNASGNWHCDSTWLGDRVITTSTRTWALPTYNNHLYKQISSASTGASNDNHYFGYSTPWGYFDFNRFHCHFSPRDWQRLINNNWGFRPKRLNFKLFNIQVKEVTTNDGVTTIANNLTSTVQVFSDSEYQLPYVLGSAHQGCLPPFPADVFMIPQYGYLTLNNGSQAVGRSSFYCLEYFPSQMLRTGNNFTFSYTFEEVPFHSSYAHSQSLDRLMNPLIDQYLYYLNRTQNQSGSAQNKDLLFSRGSPAGMSVQPKNWLPGPCYRQQRVSKTKTDNNNSNFTWTGASKYNLNGRESIINPGTAMASHKDDEDKFFPMSGVMIFGKESAGASNTALDNVMITDEEEIKATNPVATERFGTVAVNFQSSSTDPATGDVHAMGALPGMVWQDRDVYLQGPIWAKIPHTDGHFHPSPLMGGFGLKNPPPQILIKNTPVPANPPAEFSATKFASFITQYSTGQVSVEIEWELQKENSKRWNPEVQYTSNYAKSANVDFTVDNNGLYTEPRPIGTRYLTRPL

SEQ ID NO: 2 - protein, 735 aa, adeno-associated virus 2 [sequence omitted]

SEQ ID NO: 3 - protein, 736 aa, Adeno-associated virus 3A
MAADGYLPDWLEDNLSEGIREWWALKPGVPQPKANQQHQDNRRGLVLPGYKYLGPGNGLDKGEPVNEADAAALEHDKAYDQQLKAGDNPYLKYNHADAEFQERLQEDTSFGGNLGRAVFQAKKRILEPLGLVEEAAKTAPGKKGAVDQSPQEPDSSSGVGKSGKQPARKRLNFGQTGDSESVPDPQPLGEPPAAPTSLGSNTMASGGGAPMADNNEGADGVGNSSGNWHCDSQWLGDRVITTSTRTWALPTYNNHLYKQISSQSGASNDNHYFGYSTPWGYFDFNRFHCHFSPRDWQRLINNNWGFRPKKLSFKLFNIQVRGVTQNDGTTTIANNLTSTVQVFTDSEYQLPYVLGSAHQGCLPPFPADVFMVPQYGYLTLNNGSQAVGRSSFYCLEYFPSQMLRTGNNFQFSYTFEDVPFHSSYAHSQSLDRLMNPLIDQYLYYLNRTQGTTSGTTNQSRLLFSQAGPQSMSLQARNWLPGPCYRQQRLSKTANDNNNSNFPWTAASKYHLNGRDSLVNPGPAMASHKDDEEKFFPMHGNLIFGKEGTTASNAELDNVMITDEEEIRTTNPVATEQYGTVANNLQSSNTAPTTGTVNHQGALPGMVWQDRDVYLQGPIWAKIPHTDGHFHPSPLMGGFGLKHPPPQIMIKNTPVPANPPTTFSPAKFASFITQYSTGQVSVEIEWELQKENSKRWNPEIQYTSNYNKSVNVDFTVDTNGVYSEPRPIGTRYLTRNL

SEQ ID NO: 4 - protein, 736 aa, Adeno-associated virus 3B
MAADGYLPDWLEDNLSEGIREWWALKPGVPQPKANQQHQDNRRGLVLPGYKYLGPGNGLDKGEPVNEADAAALEHDKAYDQQLKAGDNPYLKYNHADAEFQERLQEDTSFGGNLGRAVFQAKKRILEPLGLVEEAAKTAPGKKRPVDQSPQEPDSSSGVGKSGKQPARKRLNFGQTGDSESVPDPQPLGEPPAAPTSLGSNTMASGGGAPMADNNEGADGVGNSSGNWHCDSQWLGDRVITTSTRTWALPTYNNHLYKQISSQSGASNDNHYFGYSTPWGYFDFNRFHCHFSPRDWQRLINNNWGFRPKKLSFKLFNIQVKEVTQNDGTTTIANNLTSTVQVFTDSEYQLPYVLGSAHQGCLPPFPADVFMVPQYGYLTLNNGSQAVGRSSFYCLEYFPSQMLRTGNNFQFSYTFEDVPFHSSYAHSQSLDRLMNPLIDQYLYYLNRTQGTTSGTTNQSRLLFSQAGPQSMSLQARNWLPGPCYRQQRLSKTANDNNNSNFPWTAASKYHLNGRDSLVNPGPAMASHKDDEEKFFPMHGNLIFGKEGTTASNAELDNVMITDEEEIRTTNPVATEQYGTVANNLQSSNTAPTTRTVNDQGALPGMVWQDRDVYLQGPIWAKIPHTDGHFHPSPLMGGFGLKHPPPQIMIKNTPVPANPPTTFSPAKFASFITQYSTGQVSVEIEWELQKENSKRWNPEIQYTSNYNKSVNVDFTVDTNGVYSEPRPIGTRYLTRNL

SEQ ID NO: 5 - protein, 734 aa, Adeno-associated virus 4
MTDGYLPDWLEDNLSEGVREWWALQPGAPKPKANQQHQDNARGLVLPGYKYLGPGNGLDKGEPVNAADAAALEHDKAYDQQLKAGDNPYLKYNHADAEFQQRLQGDTSFGGNLGRAVFQAKKRVLEPLGLVEQAGETAPGKKRPLIESPQQPDSSTGIGKKGKQPAKKKLVFEDETGAGDGPPEGSTSGAMSDDSEMRAAAGGAAVEGGQGADGVGNASGDWHCDSTWSEGHVTTTSTRTWVLPTYNNHLYKRLGESLQSNTYNGFSTPWGYFDFNRFHCHFSPRDWQRLINNNWGMRPKAMRVKIFNIQVKEVTTSNGETTVANNLTSTVQIFADSSYELPYVMDAGQEGSLPPFPNDVFMVPQYGYCGLVTGNTSQQQTDRNAFYCLEYFPSQMLRTGNNFEITYSFEKVPFHSMYAHSQSLDRLMNPLIDQYLWGLQSTTTGTTLNAGTATTNFTKLRPTNFSNFKKNWLPGPSIKQQGFSKTANQNYKIPATGSDSLIKYETHSTLDGRWSALTPGPPMATAGPADSKFSNSQLIFAGPKQNGNTATVPGTLIFTSEEELAATNATDTDMWGNLPGGDQSNSNLPTVDRLTALGAVPGMVWQNRDIYYQGPIWAKIPHTDGHFHPSPLIGGFGLKHPPPQIFIKNTPVPANPATTFSSTPVNSFITQYSTGQVSVQIDWEIQKERSKRWNPEVQFTSNYGQQNSLLWAPDAAGKYTEPRAIGTRYLTHHL

SEQ ID NO: 6 - protein, 724 aa, Adeno-associated virus 5
MSFVDHPPDWLEEVGEGLREFLGLEAGPPKPKPNQQHQDQARGLVLPGYNYLGPGNGLDRGEPVNRADEVAREHDISYNEQLEAGDNPYLKYNHADAEFQEKLADDTSFGGNLGKAVFQAKKRVLEPFGLVEEGAKTAPTGKRIDDHFPKRKKARTEEDSKPSTSSDAEAGPSGSQQLQIPAQPASSLGADTMSAGGGGPLGDNNQGADGVGNASGDWHCDSTWMGDRVVTKSTRTWVLPSYNNHQYREIKSGSVDGSNANAYFGYSTPWGYFDFNRFHSHWSPRDWQRLINNYWGFRPRSLRVKIFNIQVKEVTVQDSTTTIANNLTSTVQVFTDDDYQLPYVVGNGTEGCLPAFPPQVFTLPQYGYATLNRDNTENPTERSSFFCLEYFPSKMLRTGNNFEFTYNFEEVPFHSSFAPSQNLFKLANPLVDQYLYRFVSTNNTGGVQFNKNLAGRYANTYKNWFPGPMGRTQGWNLGSGVNRASVSAFATTNRMELEGASYQVPPQPNGMTNNLQGSNTYALENTMIFNSQPANPGTTATYLEGNMLITSESETQPVNRVAYNVGGQMATNNQSSTTAPATGTYNLQEIVPGSVWMERDVYLQGPIWAKIPETGAHFHPSPAMGGFGLKHPPPMMLIKNTPVPGNITSFSDVPVSSFITQYSTGQVTVEMEWELKKENSKRWNPEIQYTNNYNDPQFVDFAPDSTGEYRTTRPIGTRYLTRPL

SEQ ID NO: 7 - protein, 736 aa, Adeno-associated virus 6
MAADGYLPDWLEDNLSEGIREWWDLKPGAPKPKANQQKQDDGRGLVLPGYKYLGPFNGLDKGEPVNAADAAALEHDKAYDQQLKAGDNPYLRYNHADAEFQERLQEDTSFGGNLGRAVFQAKKRVLEPFGLVEEGAKTAPGKKRPVEQSPQEPDSSSGIGKTGQQPAKKRLNFGQTGDSESVPDPQPLGEPPATPAAVGPTTMASGGGAPMADNNEGADGVGNASGNWHCDSTWLGDRVITTSTRTWALPTYNNHLYKQISSASTGASNDNHYFGYSTPWGYFDFNRFHCHFSPRDWQRLINNNWGFRPKRLNFKLFNIQVKEVTTNDGVTTIANNLTSTVQVFSDSEYQLPYVLGSAHQGCLPPFPADVFMIPQYGYLTLNNGSQAVGRSSFYCLEYFPSQMLRTGNNFTFSYTFEDVPFHSSYAHSQSLDRLMNPLIDQYLYYLNRTQNQSGSAQNKDLLFSRGSPAGMSVQPKNWLPGPCYRQQRVSKTKTDNNNSNFTWTGASKYNLNGRESIINPGTAMASHKDDKDKFFPMSGVMIFGKESAGASNTALDNVMITDEEEIKATNPVATERFGTVAVNLQSSSTDPATGDVHVMGALPGMVWQDRDVYLQGPIWAKIPHTDGHFHPSPLMGGFGLKHPPPQILIKNTPVPANPPAEFSATKFASFITQYSTGQVSVEIEWELQKENSKRWNPEVQYTSNYAKSANVDFTVDNNGLYTEPRPIGTRYLTRPL

SEQ ID NO: 8 - protein, 737 aa, Adeno-associated virus 7
MAADGYLPDWLEDNLSEGIREWWDLKPGAPKPKANQQKQDNGRGLVLPGYKYLGPFNGLDKGEPVNAADAAALEHDKAYDQQLKAGDNPYLRYNHADAEFQERLQEDTSFGGNLGRAVFQAKKRVLEPLGLVEEGAKTAPAKKRPVEPSPQRSPDSSTGIGKKGQQPARKRLNFGQTGDSESVPDPQPLGEPPAAPSSVGSGTVAAGGGAPMADNNEGADGVGNASGNWHCDSTWLGDRVITTSTRTWALPTYNNHLYKQISSETAGSTNDNTYFGYSTPWGYFDFNRFHCHFSPRDWQRLINNNWGFRPKKLRFKLFNIQVKEVTTNDGVTTIANNLTSTIQVFSDSEYQLPYVLGSAHQGCLPPFPADVFMIPQYGYLTLNNGSQSVGRSSFYCLEYFPSQMLRTGNNFEFSYSFEDVPFHSSYAHSQSLDRLMNPLIDQYLYYLARTQSNPGGTAGNRELQFYQGGPSTMAEQAKNWLPGPCFRQQRVSKTLDQNNNSNFAWTGATKYHLNGRNSLVNPGVAMATHKDDEDRFFPSSGVLIFGKTGATNKTTLENVLMTNEEEIRPTNPVATEEYGIVSSNLQAANTAAQTQVVNNQGALPGMVWQNRDVYLQGPIWAKIPHTDGNFHPSPLMGGFGLKHPPPQILIKNTPVPANPPEVFTPAKFASFITQYSTGQVSVEIEWELQKENSKRWNPEIQYTSNFEKQTGVDFAVDSQGVYSEPRPIGTRYLTRNL

SEQ ID NO: 9 - protein, 738 aa, Adeno-associated virus 8
MAADGYLPDWLEDNLSEGIREWWALKPGAPKPKANQQKQDDGRGLVLPGYKYLGPFNGLDKGEPVNAADAAALEHDKAYDQQLQAGDNPYLRYNHADAEFQERLQEDTSFGGNLGRAVFQAKKRVLEPLGLVEEGAKTAPGKKRPVEPSPQRSPDSSTGIGKKGQQPARKRLNFGQTGDSESVPDPQPLGEPPAAPSGVGPNTMAAGGGAPMADNNEGADGVGSSSGNWHCDSTWLGDRVITTSTRTWALPTYNNHLYKQISNGTSGGATNDNTYFGYSTPWGYFDFNRFHCHFSPRDWQRLINNNWGFRPKRLSFKLFNIQVKEVTQNEGTKTIANNLTSTIQVFTDSEYQLPYVLGSAHQGCLPPFPADVFMIPQYGYLTLNNGSQAVGRSSFYCLEYFPSQMLRTGNNFQFTYTFEDVPFHSSYAHSQSLDRLMNPLIDQYLYYLSRTQTTGGTANTQTLGFSQGGPNTMANQAKNWLPGPCYRQQRVSTTTGQNNNSNFAWTAGTKYHLNGRNSLANPGIAMATHKDDEERFFPSNGILIFGKQNAARDNADYSDVMLTSEEEIKTTNPVATEEYGIVADNLQQQNTAPQIGTVNSQGALPGMVWQNRDVYLQGPIWAKIPHTDGNFHPSPLMGGFGLKHPPPQILIKNTPVPADPPTTFNQSKLNSFITQYSTGQVSVEIEWELQKENSKRWNPEIQYTSNYYKSTSVDFAVNTEGVYSEPRPIGTRYLTRNL

SEQ ID NO: 10 - protein, 736 aa, Adeno-associated virus 9
MAADGYLPDWLEDNLSEGIREWWALKPGAPQPKANQQHQDNARGLVLPGYKYLGPGNGLDKGEPVNAADAAALEHDKAYDQQLKAGDNPYLKYNHADAEFQERLKEDTSFGGNLGRAVFQAKKRLLEPLGLVEEAAKTAPGKKRPVEQSPQEPDSSAGIGKSGAQPAKKRLNFGQTGDTESVPDPQPIGEPPAAPSGVGSLTMASGGGAPVADNNEGADGVGSSSGNWHCDSQWLGDRVITTSTRTWALPTYNNHLYKQISNSTSGGSSNDNAYFGYSTPWGYFDFNRFHCHFSPRDWQRLINNNWGFRPKRLNFKLFNIQVKEVTDNNGVKTIANNLTSTVQVFTDSDYQLPYVLGSAHEGCLPPFPADVFMIPQYGYLTLNDGSQAVGRSSFYCLEYFPSQMLRTGNNFQFSYEFENVPFHSSYAHSQSLDRLMNPLIDQYLYYLSKTINGSGQNQQTLKFSVAGPSNMAVQGRNYIPGPSYRQQRVSTTVTQNNNSEFAWPGASSWALNGRNSLMNPGPAMASHKEGEDRFFPLSGSLIFGKQGTGRDNVDADKVMITNEEEIKTTNPVATESYGQVATNHQSAQAQAQTGWVQNQGILPGMVWQDRDVYLQGPIWAKIPHTDGNFHPSPLMGGFGMKHPPPQILIKNTPVPADPPTAFNKDKLNSFITQYSTGQVSVEIEWELQKENSKRWNPEIQYTSNYYKSNNVEFAVNTEGVYSEPRPIGTRYLTRNL

SEQ ID NO: 11 - protein, 738 aa, Adeno-associated virus 10
MAADGYLPDWLEDNLSEGIREWWDLKPGAPKPKANQQKQDDGRGLVLPGYKYLGPFNGLDKGEPVNAADAAALEHDKAYDQQLKAGDNPYLRYNHADAEFQERLQEDTSFGGNLGRAVFQAKKRVLEPLGLVEEAAKTAPGKKRPVEPSPQRSPDSSTGIGKKGQQPAKKRLNFGQTGESESVPDPQPIGEPPAGPSGLGSGTMAAGGGAPMADNNEGADGVGSSSGNWHCDSTWLGDRVITTSTRTWALPTYNNHLYKQISNGTSGGSTNDNTYFGYSTPWGYFDFNRFHCHFSPRDWQRLINNNWGFRPKRLSFKLFNIQVKEVTQNEGTKTIANNLTSTIQVFTDSEYQLPYVLGSAHQGCLPPFPADVFMIPQYGYLTLNNGSQAVGRSSFYCLEYFPSQMLRTGNNFEFSYTFEDVPFHSSYAHSQSLDRLMNPLIDQYLYYLSRTQSTGGTQGTQQLLFSQAGPANMSAQAKNWLPGPCYRQQRVSTTLSQNNNSNFAWTGATKYHLNGRDSLVNPGVAMATHKDDEERFFPSSGVLMFGKQGAGRDNVDYSSVMLTSEEEIKTTNPVATEQYGVVADNLQQANTGPIVGNVNSQGALPGMVWQNRDVYLQGPIWAKIPHTDGNFHPSPLMGGFGLKHPPPQILIKNTPVPADPPTTFSQAKLASFITQYSTGQVSVEIEWELQKENSKRWNPEIQYTSNYYKSTNVDFAVNTEGTYSEPRPIGTRYLTRNL

SEQ ID NO: 12 - protein, 738 aa, Adeno-associated virus rh10
MAADGYLPDWLEDNLSEGIREWWALKPGAPKPKANQQKQDDGRGLVLPGYKYLGPFNGLDKGEPVNAADAAALEHDKAYDQQLKAGDNPYLRYNHADAEFQERLQEDTSFGGNLGRAVFQAKKRVLEPLGLVEEGAKTAPGKKRPVEPSPQRSPDSSTGIGKKGQQPAKKRLNFGQTGDSESVPDPQPIGEPPAGPSGLGSGTMAAGGGAPMADNNEGADGVGSSSGNWHCDSTWLGDGVITTSTRTWALPTYNNHLYKQISNGTSGGSTNDNTYFGYSTPWGYFDFNRFHCHFSPRDWQRLINNNWGFRPKSLNFKLFNIQVKEVTQNEGTKTIANNLTSTIQVFTDSEYQLPYVLGSAHQGCLPPFPADVFMIPQYGYLTLNNGSQAVGRSSFYCLEYFPSQMLRTGNNFEFSYQFEDVPFHSSYAHSQSLDRLMNPLIDQYLYYLSRTQSTGGTAGTQQLLFSQAGPNNMSAQAKNWLPGPCYRQQRVSTTLSQNDNSNFAWTGATKYHLNGRDSLVNPGVAMATHKDDEERFFPSSGVLMFGKQGAGKDNVDYSSVMLTSEEEIKTTNPVATEQYGVVADNLQQQNAAPIVGAVNSQGALPGMVWQNRDVYLQGPIWAKIPHTDGNFHPSPLMGGFGLKHPPPQILIKNTPVPADPPTTFSQAKLASFITQYSTGQVSVEIEWELQKENSKRWNPEIQYTSNYYKSTNVDFAVNTDGTYSEPRPIGTRYLTRNL

SEQ ID NO: 13 - protein, 7 aa, Artificial Sequence
  heterologous peptide insertion
NKIQRTD

SEQ ID NO: 14 - protein, 7 aa, Artificial Sequence
  heterologous peptide insertion
NKTTNKD

SEQ ID NO: 15 - protein, 7 aa, Artificial Sequence
  heterologous peptide insertion
TNKIGVT

SEQ ID NO: 16 - protein, 7 aa, Artificial Sequence
  heterologous peptide insertion
GNLTKGN

SEQ ID NO: 17 - protein, 7 aa, Artificial Sequence
  heterologous peptide insertion
NTVKLST

SEQ ID NO: 18 - protein, 7 aa, Artificial Sequence
  heterologous peptide insertion
SNTVKAI

SEQ ID NO: 19 - protein, 7 aa, Artificial Sequence
  heterologous peptide insertion
ASNITKA

SEQ ID NO: 20 - protein, 7 aa, Artificial Sequence
  heterologous peptide insertion
DNTVTRS

SEQ ID NO: 21 - protein, 7 aa, Artificial Sequence
  heterologous peptide insertion
NKISAKD

SEQ ID NO: 22 - protein, 7 aa, Artificial Sequence
  heterologous peptide insertion
NQDYTKT

SEQ ID NO: 23 - protein, 7 aa, Artificial Sequence
  heterologous peptide insertion
QADTTKN

SEQ ID NO: 24 - protein, 7 aa, Artificial Sequence
  heterologous peptide insertion
TNRTSPD

SEQ ID NO: 25 - protein, 7 aa, Artificial Sequence
  heterologous peptide insertion
SNTTQKT

SEQ ID NO: 26 - protein, 7 aa, Artificial Sequence
  heterologous peptide insertion
ASDSTKA

SEQ ID NO: 27 - protein, 10 aa, Artificial Sequence
  heterologous peptide insertion
LANKIQRTDA

SEQ ID NO: 28 - protein, 10 aa, Artificial Sequence
  heterologous peptide insertion
LANKTTNKDA

SEQ ID NO: 29 - protein, 10 aa, Artificial Sequence
  heterologous peptide insertion
LATNKIGVTA

SEQ ID NO: 30 - protein, 10 aa, Artificial Sequence
  heterologous peptide insertion
LAGNLTKGNA

SEQ ID NO: 31 - protein, 10 aa, Artificial Sequence
  heterologous peptide insertion
LANTVKLSTA

SEQ ID NO: 32 - protein, 10 aa, Artificial Sequence
  heterologous peptide insertion
LASNTVKAIA

SEQ ID NO: 33 - protein, 10 aa, Artificial Sequence
  heterologous peptide insertion
LAASNITKAA

SEQ ID NO: 34 - protein, 10 aa, Artificial Sequence
  heterologous peptide insertion
LADNTVTRSA

SEQ ID NO: 35 - protein, 10 aa, Artificial Sequence
  heterologous peptide insertion
LANKISAKDA

SEQ ID NO: 36 - protein, 10 aa, Artificial Sequence
  heterologous peptide insertion
LANQDYTKTA

SEQ ID NO: 37 - protein, 10 aa, Artificial Sequence
  heterologous peptide insertion
LATNKIGVTS

SEQ ID NO: 38 - protein, 10 aa, Artificial Sequence
  heterologous peptide insertion
LATNKIGVTA

SEQ ID NO: 39 - protein, 10 aa, Artificial Sequence
  heterologous peptide insertion
LAQADTTKNA

SEQ ID NO: 40 - protein, 10 aa, Artificial Sequence
  heterologous peptide insertion
LATNRTSPDA

SEQ ID NO: 41 - protein, 10 aa, Artificial Sequence
  heterologous peptide insertion
LASNTTQKTA

SEQ ID NO: 42 - protein, 10 aa, Artificial Sequence
  heterologous peptide insertion
LAASDSTKAA

SEQ ID NO: 43 - protein, 745 aa, Artificial Sequence
  variant AAV capsid
MAADGYLPDWLEDTLSEGIRQWWKLKPGPPPPKPAERHKDDSRGLVLPGYKYLGPFNGLDKGEPVNEADAAALEHDKAYDRQLDSGDNPYLKYNHADAEFQERLKEDTSFGGNLGRAVFQAKKRVLEPLGLVEEPVKTAPGKKRPVEHSPVEPDSSSGTGKAGQQPARKRLNFGQTGDADSVPDPQPLGQPPAAPSGLGTNTMATGSGAPMADNNEGADGVGNSSGNWHCDSTWMGDRVITTSTRTWALPTYNNHLYKQISSQSGASNDNHYFGYSTPWGYFDFNRFHCHFSPRDWQRLINNNWGFRPKRLNFKLFNIQVKEVTQNDGTTTIANNLTSTVQVFTDSEYQLPYVLGSAHQGCLPPFPADVFMVPQYGYLTLNNGSQAVGRSSFYCLEYFPSQMLRTGNNFTFSYTFEDVPFHSSYAHSQSLDRLMNPLIDQYLYYLSRTNTPSGTTTQSRLQFSQAGASDIRDQSRNWLPGPCYRQQRVSKTSADNNNSEYSWTGATKYHLNGRDSLVNPGPAMASHKDDEEKFFPQSGVLIFGKQGSEKTNVDIEKVMITDEEEIRTTNPVATEQYGSVSTNLQRGNLANKIQRTDARQAATADVNTQGVLPGMVWQDRDVYLQGPIWAKIPHTDGHFHPSPLMGGFGLKHPPPQILIKNTPVPANPSTTFSAAKFASFITQYSTGQVSVEIEWELQKENSKRWNPEIQYTSNYNKSINVDFTVDTNGVYSEPRPIGTRYLTRNL

SEQ ID NO: 44 - protein, 745 aa, Artificial Sequence
  variant AAV capsid
MAADGYLPDWLEDTLSEGIRQWWKLKPGPPPPKPAERHKDDSRGLVLPGYKYLGPFNGLDKGEPVNEADAAALEHDKAYDRQLDSGDNPYLKYNHADAEFQERLKEDTSFGGNLGRAVFQAKKRVLEPLGLVEEPVKTAPGKKRPVEHSPVEPDSSSGTGKAGQQPARKRLNFGQTGDADSVPDPQPLGQPPAAPSGLGTNTMATGSGAPMADNNEGADGVGNSSGNWHCDSTWMGDRVITTSTRTWALPTYNNHLYKQISSQSGASNDNHYFGYSTPWGYFDFNRFHCHFSPRDWQRLINNNWGFRPKRLKFKLFNIQVKEVTQNDGTTTIANNLTSTVQVFTDSEYQLPYVLGSAHQGCLPPFPADVFMVPQYGYLTLNNGSQAVGRSSFYCLEYFPSQMLRTGNNFTFSYTFEDVPFHSSYAHSQSLDRLMNPLIDQYLYYLSRTDTPSGTTTQSRLQFSQAGASDIRDQSRNWLPGPCYRQQRVSKTSADNNNSEYSWTGATKYHLNGRDSLVNPGPAMASHKDDEEKFFPQSGVLIFGKQGSEKTSVDIEKVMITDEEEIRTTNPVATEQYGSVSTNLQRGNLANKIQRTDARQAATADVNTQGVLPGMVWQDRDVYLQGPIWAKIPHTDGHFHPSPLMGGFGLKHPPPQILIKNTPVPANPSTTFSAAKFASFITQYSTGQVSVEIEWELQKENSKRWNPEVQYTSNYNKSVNVDFTVDTNGVYSEPRPIGTRYLTRNQ

SEQ ID NO: 45 - protein, 745 aa, Artificial Sequence
  variant AAV capsid
MAADGYLPDWLEDTLSEGIRQWWKLKPGPPPPKPAERHKDDSRGLVLPGYKYLGPFNGLDKGEPVNEADAAALEHDKAYDRQLDSGDNPYLKYNHADAEFQERLKEDTSFGGNLGRAVFQAKKRVLEPLGLVEEPVKTAPGKKRPVEHSPVEPDSSSGTGKAGQQPARKRLNFGQTGDADSVPDPQPLGQPPAAPSGLGTNTMATGSGAPMADNNEGADGVGNSSGNWHCDSTWMGDRVITTSTRTWALPTYNNHLYKQISSQSGASNDNHYFGYSTPWGYFDFNRFHCHFSPRDWQRLINNNWGFRPKRLNFKLFNIQVKEVTQNDGTTTIANNLTSTVQVFTDSEYQLPYVLGSAHQGCLPPFPADVFMVPQYGYLTLNNGSQAVGRSSFYCLEYFPSQMLRTGNNFTFSYTFEDVPFHSSYAHSQSLDRLMNPLIDQYLYYLSRTNTPSGTTTQSRLQFSQAGASDIRDQSRNWLPGPCYRQQRVSKTSADNNNSEYSWTGATKYHLNGRDSLVNPGPAMASHKDDEEKFFPQSGVLIFGKQGSEKTNVDIEKVMITDEEEIRTTNPVATEQYGSVSTNLQRGNLANKIQRTDARQAATADVNTQGVLPGMVWQDRDVYLQGPIWAKIPHTDGHFHPSPLMGGFGLKHPPPQILIKNTPVPANPSTTFSAAKFASFITQYSTGQVSVEIEWELQKENSKRWNPEIQYTSNYNKSVNVDFTVDTNGVYSEPRPIGTRYLTRNL

SEQ ID NO: 46 - protein, 745 aa, Artificial Sequence
  variant AAV capsid
MAADGYLPDWLEDTLSEGIRQWWKLKPGPPPPKPAERHKDDSRGLVLPGYKYLGPFNGLDKGEPVNEADAAALEHDKAYDRQLDSGDNPYLKYNHADAEFQERLKEDTSFGGNLGRAVFQAKKRVLEPLGLVEEPVKTAPGKKRPVEHSPVEPDSSSGTGKAGQQPARKRLNFGQTGDADSVPDPQPLGQPPAAPSGLGTNTMATGSGAPMADNNEGADGVGNSSGNWHCDSTWMGDRVITTSTRTWALPTYNNHLYKQISSQSGASNDNHYFGYSTPWGYFDFNRFHCHFSPRDWQRLINNNWGFRPKRLNFKLFNIQVKEVTQNDGTTTIANNLTSTVQVFTDSEYQLPYVLGSAHQGCLPPFPADVFMVPQYGYLTLNNGSQAVGRSSFYCLEYFPSQMLRTGNNFTFSYTFEDVPFHSSYAHSQSLDRLMNPLIDQYLYYLSRTNTPSGTTTQSRLQFSQAGASDIRDQSRNWLPGPCYRQQRVSKTSADNNNSEYSWTGATKYHLNGRDSLVNPGPAMASHKDDEEKFFPQSGVLIFGKQGSEKTNVDIEKVMITDEEEIRTTNPVATEQYGSVSTNLQRGNLATNKIGVTARQAATADVNTQGVLPGMVWQDRDVYLQGPIWAKIPHTDGHFHPSPLMGGFGLKHPPPQILIKNTPVPANPSTTFSAAKFASFITQYSTGQVSVEIEWELQKENSKRWNPEIQYTSNYNKSINVDFTVDTNGVYSEPRPIGTRYLTRNL

SEQ ID NO: 47 - protein, 745 aa, Artificial Sequence
  variant AAV capsid
MAADGYLPDWLEDTLSEGIRQWWKLKPGPPPPKPAERHKDDSRGLVLPGYKYLGPFNGLDKGEPVNEADAAALEHDKAYDRQLDSGDNPYLKYNHADAEFQERLKEDTSFGGNLGRAVFQAKKRVLEPLGLVEEPVKTAPGKKRPVEHSPVEPDSSSGTGKAGQQPARKRLNFGQTGDADSVPDPQPLGQPPAAPSGLGTNTMATGSGAPMADNNEGADGVGNSSGNWHCDSTWMGDRVITTSTRTWALPTYNNHLYKQISSQSGASNDNHYFGYSTPWGYFDFNRFHCHFSPRDWQRLINNNWGFRPKRLNFKLFNIQVKEVTQNDGTTTIANNLTSTVQVFTDSEYQLPYVLGSAHQGCLPPFPADVFMVPQYGYLTLNNGSQAVGRSSFYCLEYFPSQMLRTGNNFTFSYTFEDVPFHSSYAHSQSLDRLMNPLIDQYLYYLSRTNTPSGTTTQSRLQFSQAGASDIRDQSRNWLPGPCYRQQRVSKTSADNNNSEYSWTGATKYHLNGRDSLVNPGPAMASHKDDEEKFFPQSGVLIFGKQGSEKTNVDIEKVMITDEEEIRTTNPVATEQYGSVSTNLQRGNLATNKIGVTARQAATADVNTQGVLPGMVWQDRDVYLQGPIWAKIPHTDGHFHPSPLMGGFGLKHPPPQILIKNTPVPANPSTTFSAAKFASFITQYSTGQVSVEIEWELQKENSKRWNPEIQYTSNYNKSVNVDFTVDTNGVYSEPRPIGTRYLTRNL

SEQ ID NO: 48 - protein, 745 aa, Artificial Sequence
  variant AAV capsid
MAADGYLPDWLEDTLSEGIRQWWKLKPGPPPPKPAERHKDDSRGLVLPGYKYLGPFNGLDKGEPVNEADAAALEHDKAYDRQLDSGDNPYLKYNHADAEFQERLKEDTSFGGNLGRAVFQAKKRVLEPLGLVEEPVKTAPGKKRPVEHSPVEPDSSSGTGKAGQQPARKRLNFGQTGDADSVPDPQPLGQPPAAPSGLGTNTMATGSGAPMADNNEGADGVGNSSGNWHCDSTWMGDRVITTSTRTWALPTYNNHLYKQISSQSGASNDNHYFGYSTPWGYFDFNRFHCHFSPRDWQRLINNNWGFRPKRLNFKLFNIQVKEVTQNDGTTTIANNLTSTVQVFTDSEYQLPYVLGSAHQGCLPPFPADVFMVPQYGYLTLNNGSQAVGRSSFYCLEYFPSQMLRTGNNFTFSYTFEDVPFHSSYAHSQSLDRLMNPLIDQYLYYLSRTNTPSGTTTQSRLQFSQAGASDIRDQSRNWLPGPCYRQQRVSKTSADNNNSEYSWTGATKYHLNGRDSLVNPGPAMASHKDDEEKFFPQSGVLIFGKQGSEKTNVDIEKVMITDEEEIRTTNPVATEQYGSVSTNLQRGNLANKTTNKDARQAATADVNTQGVLPGMVWQDRDVYLQGPIWAKIPHTDGHFHPSPLMGGFGLKHPPPQILIKNTPVPANPSTTFSAAKFASFITQYSTGQVSVEIEWELQKENSKRWNPEIQYTSNYNKSINVDFTVDTNGVYSEPRPIGTRYLTRNL

SEQ ID NO: 49 - protein, 745 aa, Artificial Sequence
  variant AAV capsid
MAADGYLPDWLEDTLSEGIRQWWKLKPGPPPPKPAERHKDDSRGLVLPGYKYLGPFNGLDKGEPVNEADAAALEHDKAYDRQLDSGDNPYLKYNHADAEFQERLKEDTSFGGNLGRAVFQAKKRVLEPLGLVEEPVKTAPGKKRPVEHSPVEPDSSSGTGKAGQQPARKRLNFGQTGDADSVPDPQPLGQPPAAPSGLGTNTMATGSGAPMADNNEGADGVGNSSGNWHCDSTWMGDRVITTSTRTWALPTYNNHLYKQISSQSGASNDNHYFGYSTPWGYFDFNRFHCHFSPRDWQRLINNNWGFRPKRLKFKLFNIQVKEVTQNDGTTTIANNLTSTVQVFTDSEYQLPYVLGSAHQGCLPPFPADVFMVPQYGYLTLNNGSQAVGRSSFYCLEYFPSQMLRTGNNFTFSYTFEDVPFHSSYAHSQSLDRLMNPLIDQYLYYLSRTDTPSGTTTQSRLQFSQAGASDIRDQSRNWLPGPCYRQQRVSKTSADNNNSEYSWTGATKYHLNGRDSLVNPGPAMASHKDDEEKFFPQSGVLIFGKQGSEKTSVDIEKVMITDEEEIRTTNPVATEQYGSVSTNLQRGNLANKTTNKDARQAATADVNTQGVLPGMVWQDRDVYLQGPIWAKIPHTDGHFHPSPLMGGFGLKHPPPQILIKNTPVPANPSTTFSAAKFASFITQYSTGQVSVEIEWELQKENSKRWNPEVQYTSNYNKSVNVDFTVDTNGVYSEPRPIGTRYLTRNQ

SEQ ID NO: 50 - protein, 745 aa, Artificial Sequence
  variant AAV capsid
MAADGYLPDWLEDTLSEGIRQWWKLKPGPPPPKPAERHKDDSRGLVLPGYKYLGPFNGLDKGEPVNEADAAALEHDKAYDRQLDSGDNPYLKYNHADAEFQERLKEDTSFGGNLGRAVFQAKKRVLEPLGLVEEPVKTAPGKKRPVEHSPVEPDSSSGTGKAGQQPARKRLNFGQTGDADSVPDPQPLGQPPAAPSGLGTNTMATGSGAPMADNNEGADGVGNSSGNWHCDSTWMGDRVITTSTRTWALPTYNNHLYKQISSQSGASNDNHYFGYSTPWGYFDFNRFHCHFSPRDWQRLINNNWGFRPKRLNFKLFNIQVKEVTQNDGTTTIANNLTSTVQVFTDSEYQLPYVLGSAHQGCLPPFPADVFMVPQYGYLTLNNGSQAVGRSSFYCLEYFPSQMLRTGNNFTFSYTFEDVPFHSSYAHSQSLDRLMNPLIDQYLYYLSRTNTPSGTTTQSRLQFSQAGASDIRDQSRNWLPGPCYRQQRVSKTSADNNNSEYSWTGATKYHLNGRDSLVNPGPAMASHKDDEEKFFPQSGVLIFGKQGSEKTNVDIEKVMITDEEEIRTTNPVATEQYGSVSTNLQRGNLANKTTNKDARQAATADVNTQGVLPGMVWQDRDVYLQGPIWAKIPHTDGHFHPSPLMGGFGLKHPPPQILIKNTPVPANPSTTFSAAKFASFITQYSTGQVSVEIEWELQKENSKRWNPEIQYTSNYNKSVNVDFTVDTNGVYSEPRPIGTRYLTRNL

SEQ ID NO: 51 - protein, 745 aa, Artificial Sequence
  variant AAV capsid
MAADGYLPDWLEDTLSEGIRQWWKLKPGPPPPKPAERHKDDSRGLVLPGYKYLGPFNGLDKGEPVNEADAAALEHDKAYDRQLDSGDNPYLKYNHADAEFQERLKEDTSFGGNLGRAVFQAKKRVLEPLGLVEEPVKTAPGKKRPVEHSPVEPDSSSGTGKAGQQPARKRLNFGQTGDADSVPDPQPLGQPPAAPSGLGTNTMATGSGAPMADNNEGADGVGNSSGNWHCDSTWMGDRVITTSTRTWALPTYNNHLYKQISSQSGASNDNHYFGYSTPWGYFDFNRFHCHFSPRDWQRLINNNWGFRPKRLNFKLFNIQVKEVTQNDGTTTIANNLTSTVQVFTDSEYQLPYVLGSAHQGCLPPFPADVFMVPQYGYLTLNNGSQAVGRSSFYCLEYFPSQMLRTGNNFTFSYTFEDVPFHSSYAHSQSLDRLMNPLIDQYLYYLSRTNTPSGTTTQSRLQFSQAGASDIRDQSRNWLPGPCYRQQRVSKTSADNNNSEYSWTGATKYHLNGRDSLVNPGPAMASHKDDEEKFFPQSGVLIFGKQGSEKTNVDIEKVMITDEEEIRTTNPVATEQYGSVSTNLQRGNLAGNLTKGNARQAATADVNTQGVLPGMVWQDRDVYLQGPIWAKIPHTDGHFHPSPLMGGFGLKHPPPQILIKNTPVPANPSTTFSAAKFASFITQYSTGQVSVEIEWELQKENSKRWNPEIQYTSNYNKSVNVDFTVDTNGVYSEPRPIGTRYLTRNL

SEQ ID NO: 52 - protein, 745 aa, Artificial Sequence
  variant AAV capsid
MAADGYLPDWLEDTLSEGIRQWWKLKPGPPPPKPAERHKDDSRGLVLPGYKYLGPFNGLDKGEPVNEADAAALEHDKAYDRQLDSGDNPYLKYNHADAEFQERLKEDTSFGGNLGRAVFQAKKRVLEPLGLVEEPVKTAPGKKRPVEHSPVEPDSSSGTGKAGQQPARKRLNFGQTGDADSVPDPQPLGQPPAAPSGLGTNTMATGSGAPMADNNEGADGVGNSSGNWHCDSTWMGDRVITTSTRTWALPTYNNHLYKQISSQSGASNDNHYFGYSTPWGYFDFNRFHCHFSPRDWQRLINNNWGFRPKRLNFKLFNIQVKEVTQNDGTTTIANNLTSTVQVFTDSEYQLPYVLGSAHQGCLPPFPADVFMVPQYGYLTLNNGSQAVGRSSFYCLEYFPSQMLRTGNNFTFSYTFEDVPFHSSYAHSQSLDRLMNPLIDQYLYYLSRTNTPSGTTTQSRLQFSQAGASDIRDQSRNWLPGPCYRQQRVSKTSADNNNSEYSWTGATKYHLNGRDSLVNPGPAMASHKDDEEKFFPQSGVLIFGKQGSEKTNVDIEKVMITDEEEIRTTNPVATEQYGSVSTNLQRGNLANTVKLSTARQAATADVNTQGVLPGMVWQDRDVYLQGPIWAKIPHTDGHFHPSPLMGGFGLKHPPPQILIKNTPVPANPSTTFSAAKFASFITQYSTGQVSVEIEWELQKENSKRWNPEIQYTSNYNKSVNVDFTVDTNGVYSEPRPIGTRYLTRNL

SEQ ID NO: 53 - protein, 745 aa, Artificial Sequence
  variant AAV capsid
MAADGYLPDWLEDTLSEGIRQWWKLKPGPPPPKPAERHKDDSRGLVLPGYKYLGPFNGLDKGEPVNEADAAALEHDKAYDRQLDSGDNPYLKYNHADAEFQERLKEDTSFGGNLGRAVFQAKKRVLEPLGLVEEPVKTAPGKKRPVEHSPVEPDSSSGTGKAGQQPARKRLNFGQTGDADSVPDPQPLGQPPAAPSGLGTNTMATGSGAPMADNNEGADGVGNSSGNWHCDSTWMGDRVITTSTRTWALPTYNNHLYKQISSQSGASNDNHYFGYSTPWGYFDFNRFHCHFSPRDWQRLINNNWGFRPKRLNFKLFNIQVKEVTQNDGTTTIANNLTSTVQVFTDSEYQLPYVLGSAHQGCLPPFPADVFMVPQYGYLTLNNGSQAVGRSSFYCLEYFPSQMLRTGNNFTFSYTFEDVPFHSSYAHSQSLDRLMNPLIDQYLYYLSRTNTPSGTTTQSRLQFSQAGASDIRDQSRNWLPGPCYRQQRVSKTSADNNNSEYSWTGATKYHLNGRDSLVNPGPAMASHKDDEEKFFPQSGVLIFGKQGSEKTNVDIEKVMITDEEEIRTTNPVATEQYGSVSTNLQRGNLASNTVKAIARQAATADVNTQGVLPGMVWQDRDVYLQGPIWAKIPHTDGHFHPSPLMGGFGLKHPPPQILIKNTPVPANPSTTFSAAKFASFITQYSTGQVSVEIEWELQKENSKRWNPEIQYTSNYNKSVNVDFTVDTNGVYSEPRPIGTRYLTRNL

SEQ ID NO: 54 - protein, 745 aa, Artificial Sequence
  variant AAV capsid
MAADGYLPDWLEDTLSEGIRQWWKLKPGPPPPKPAERHKDDSRGLVLPGYKYLGPFNGLDKGEPVNEADAAALEHDKAYDRQLDSGDNPYLKYNHADAEFQERLKEDTSFGGNLGRAVFQAKKRVLEPLGLVEEPVKTAPGKKRPVEHSPVEPDSSSGTGKAGQQPARKRLNFGQTGDADSVPDPQPLGQPPAAPSGLGTNTMATGSGAPMADNNEGADGVGNSSGNWHCDSTWMGDRVITTSTRTWALPTYNNHLYKQISSQSGASNDNHYFGYSTPWGYFDFNRFHCHFSPRDWQRLINNNWGFRPKRLNFKLFNIQVKEVTQNDGTTTIANNLTSTVQVFTDSEYQLPYVLGSAHQGCLPPFPADVFMVPQYGYLTLNNGSQAVGRSSFYCLEYFPSQMLRTGNNFTFSYTFEDVPFHSSYAHSQSLDRLMNPLIDQYLYYLSRTNTPSGTTTQSRLQFSQAGASDIRDQSRNWLPGPCYRQQRVSKTSADNNNSEYSWTGATKYHLNGRDSLVNPGPAMASHKDDEEKFFPQSGVLIFGKQGSEKTNVDIEKVMITDEEEIRTTNPVATEQYGSVSTNLQRGNLAASNITKAARQAATADVNTQGVLPGMVWQDRDVYLQGPIWAKIPHTDGHFHPSPLMGGFGLKHPPPQILIKNTPVPANPSTTFSAAKFASFITQYSTGQVSVEIEWELQKENSKRWNPEIQYTSNYNKSVNVDFTVDTNGVYSEPRPIGTRYLTRNL

SEQ ID NO: 55 - protein, 745 aa, Artificial Sequence
  variant AAV capsid
MAADGYLPDWLEDTLSEGIRQWWKLKPGPPPPKPAERHKDDSRGLVLPGYKYLGPFNGLDKGEPVNEADAAALEHDKAYDRQLDSGDNPYLKYNHADAEFQERLKEDTSFGGNLGRAVFQAKKRVLEPLGLVEEPVKTAPGKKRPVEHSPVEPDSSSGTGKAGQQPARKRLNFGQTGDADSVPDPQPLGQPPAAPSGLGTNTMATGSGAPMADNNEGADGVGNSSGNWHCDSTWMGDRVITTSTRTWALPTYNNHLYKQISSQSGASNDNHYFGYSTPWGYFDFNRFHCHFSPRDWQRLINNNWGFRPKRLNFKLFNIQVKEVTQNDGTTTIANNLTSTVQVFTDSEYQLPYVLGSAHQGCLPPFPADVFMVPQYGYLTLNNGSQAVGRSSFYCLEYFPSQMLRTGNNFTFSYTFEDVPFHSSYAHSQSLDRLMNPLIDQYLYYLSRTNTPSGTTTQSRLQFSQAGASDIRDQSRNWLPGPCYRQQRVSKTSADNNNSEYSWTGATKYHLNGRDSLVNPGPAMASHKDDEEKFFPQSGVLIFGKQGSEKTNVDIEKVMITDEEEIRTTNPVATEQYGSVSTNLQRGNLADNTVTRSARQAATADVNTQGVLPGMVWQDRDVYLQGPIWAKIPHTDGHFHPSPLMGGFGLKHPPPQILIKNTPVPANPSTTFSAAKFASFITQYSTGQVSVEIEWELQKENSKRWNPEIQYTSNYNKSVNVDFTVDTNGVYSEPRPIGTRYLTRNL

SEQ ID NO: 56 - protein, 745 aa, Artificial Sequence
  variant AAV capsid
MAADGYLPDWLEDTLSEGIRQWWKLKPGPPPPKPAERHKDDSRGLVLPGYKYLGPFNGLDKGEPVNEADAAALEHDKAYDRQLDSGDNPYLKYNHADAEFQERLKEDTSFGGNLGRAVFQAKKRVLEPLGLVEEPVKTAPGKKRPVEHSPVEPDSSSGTGKAGQQPARKRLNFGQTGDADSVPDPQPLGQPPAAPSGLGTNTMATGSGAPMADNNEGADGVGNSSGNWHCDSTWMGDRVITTSTRTWALPTYNNHLYKQISSQSGASNDNHYFGYSTPWGYFDFNRFHCHFSPRDWQRLINNNWGFRPKRLNFKLFNIQVKEVTQNDGTTTIANNLTSTVQVFTDSEYQLPYVLGSAHQGCLPPFPADVFMVPQYGYLTLNNGSQAVGRSSFYCLEYFPSQMLRTGNNFTFSYTFEDVPFHSSYAHSQSLDRLMNPLIDQYLYYLSRTNTPSGTTTQSRLQFSQAGASDIRDQSRNWLPGPCYRQQRVSKTSADNNNSEYSWTGATKYHLNGRDSLVNPGPAMASHKDDEEKFFPQSGVLIFGKQGSEKTNVDIEKVMITDEEEIRTTNPVATEQYGSVSTNLQRGNLANKISAKDARQAATADVNTQGVLPGMVWQDRDVYLQGPIWAKIPHTDGHFHPSPLMGGFGLKHPPPQILIKNTPVPANPSTTFSAAKFASFITQYSTGQVSVEIEWELQKENSKRWNPEIQYTSNYNKSVNVDFTVDTNGVYSEPRPIGTRYLTRNL

SEQ ID NO: 57 - protein, 745 aa, Artificial Sequence
  variant AAV capsid
MAADGYLPDWLEDTLSEGIRQWWKLKPGPPPPKPAERHKDDSRGLVLPGYKYLGPFNGLDKGEPVNEADAAALEHDKAYDRQLDSGDNPYLKYNHADAEFQERLKEDTSFGGNLGRAVFQAKKRVLEPLGLVEEPVKTAPGKKRPVEHSPVEPDSSSGTGKAGQQPARKRLNFGQTGDADSVPDPQPLGQPPAAPSGLGTNTMATGSGAPMADNNEGADGVGNSSGNWHCDSTWMGDRVITTSTRTWALPTYNNHLYKQISSQSGASNDNHYFGYSTPWGYFDFNRFHCHFSPRDWQRLINNNWGFRPKRLNFKLFNIQVKEVTQNDGTTTIANNLTSTVQVFTDSEYQLPYVLGSAHQGCLPPFPADVFMVPQYGYLTLNNGSQAVGRSSFYCLEYFPSQMLRTGNNFTFSYTFEDVPFHSSYAHSQSLDRLMNPLIDQYLYYLSRTNTPSGTTTQSRLQFSQAGASDIRDQSRNWLPGPCYRQQRVSKTSADNNNSEYSWTGATKYHLNGRDSLVNPGPAMASHKDDEEKFFPQSGVLIFGKQGSEKTNVDIEKVMITDEEEIRTTNPVATEQYGSVSTNLQRGNLANQDYTKTARQAATADVNTQGVLPGMVWQDRDVYLQGPIWAKIPHTDGHFHPSPLMGGFGLKHPPPQILIKNTPVPANPSTTFSAAKFASFITQYSTGQVSVEIEWELQKENSKRWNPEIQYTSNYNKSVNVDFTVDTNGVYSEPRPIGTRYLTRNL

SEQ ID NO: 58 - protein, 745 aa, Artificial Sequence
  variant AAV capsid
MAADGYLPDWLEDTLSEGIRQWWKLKPGPPPPKPAERHKDDSRGLVLPGYKYLGPFNGLDKGEPVNEADAAALEHDKAYDRQLDSGDNPYLKYNHADAEFQERLKEDTSFGGNLGRAVFQAKKRVLEPLGLVEEPVKTAPGKKRPVEHSPVEPDSSSGTGKAGQQPARKRLNFGQTGDADSVPDPQPLGQPPAAPSGLGTNTMATGSGAPMADNNEGADGVGNSSGNWHCDSTWMGDRVITTSTRTWALPTYNNHLYKQISSQSGASNDNHYFGYSTPWGYFDFNRFHCHFSPRDWQRLINNNWGFRPKRLNFKLFNIQVKEVTQNDGTTTIANNLTSTVQVFTDSEYQLPYVLGSAHQGCLPPFPADVFMVPQYGYLTLNNGSQAVGRSSFYCLEYFPSQMLRTGNNFTFSYTFEDVPFHSSYAHSQSLDRLMNPLIDQYLYYLSRTNTPSGTTTQSRLQFSQAGASDIRDQSRNWLPGPCYRQQRVSKTSADNNNSEYSWTGATKYHLNGRDSLVNPGPAMASHKDDEEKFFPQSGVLIFGKQGSEKTNVDIEKVMITDEEEIRTTNPVATEQYGSVSTNLQRGNLAQADTTKNARQAATADVNTQGVLPGMVWQDRDVYLQGPIWAKIPHTDGHFHPSPLMGGFGLKHPPPQILIKNTPVPANPSTTFSAAKFASFITQYSTGQVSVEIEWELQKENSKRWNPEIQYTSNYNKSVNVDFTVDTNGVYSEPRPIGTRYLTRNL

SEQ ID NO: 59 - protein, 745 aa, Artificial Sequence
  variant AAV capsid
MAADGYLPDWLEDTLSEGIRQWWKLKPGPPPPKPAERHKDDSRGLVLPGYKYLGPFNGLDKGEPVNEADAAALEHDKAYDRQLDSGDNPYLKYNHADAEFQERLKEDTSFGGNLGRAVFQAKKRVLEPLGLVEEPVKTAPGKKRPVEHSPVEPDSSSGTGKAGQQPARKRLNFGQTGDADSVPDPQPLGQPPAAPSGLGTNTMATGSGAPMADNNEGADGVGNSSGNWHCDSTWMGDRVITTSTRTWALPTYNNHLYKQISSQSGASNDNHYFGYSTPWGYFDFNRFHCHFSPRDWQRLINNNWGFRPKRLNFKLFNIQVKEVTQNDGTTTIANNLTSTVQVFTDSEYQLPYVLGSAHQGCLPPFPADVFMVPQYGYLTLNNGSQAVGRSSFYCLEYFPSQMLRTGNNFTFSYTFEDVPFHSSYAHSQSLDRLMNPLIDQYLYYLSRTNTPSGTTTQSRLQFSQAGASDIRDQSRNWLPGPCYRQQRVSKTSADNNNSEYSWTGATKYHLNGRDSLVNPGPAMASHKDDEEKFFPQSGVLIFGKQGSEKTNVDIEKVMITDEEEIRTTNPVATEQYGSVSTNLQRGNLATNRTSPDARQAATADVNTQGVLPGMVWQDRDVYLQGPIWAKIPHTDGHFHPSPLMGGFGLKHPPPQILIKNTPVPANPSTTFSAAKFASFITQYSTGQVSVEIEWELQKENSKRWNPEIQYTSNYNKSINVDFTVDTNGVYSEPRPIGTRYLTRNL

SEQ ID NO: 60 - protein, 745 aa, Artificial Sequence
  variant AAV capsid
MAADGYLPDWLEDTLSEGIRQWWKLKPGPPPPKPAERHKDDSRGLVLPGYKYLGPFNGLDKGEPVNEADAAALEHDKAYDRQLDSGDNPYLKYNHADAEFQERLKEDTSFGGNLGRAVFQAKKRVLEPLGLVEEPVKTAPGKKRPVEHSPVEPDSSSGTGKAGQQPARKRLNFGQTGDADSVPDPQPLGQPPAAPSGLGTNTMATGSGAPMADNNEGADGVGNSSGNWHCDSTWMGDRVITTSTRTWALPTYNNHLYKQISSQSGASNDNHYFGYSTPWGYFDFNRFHCHFSPRDWQRLINNNWGFRPKRLNFKLFNIQVKEVTQNDGTTTIANNLTSTVQVFTDSEYQLPYVLGSAHQGCLPPFPADVFMVPQYGYLTLNNGSQAVGRSSFYCLEYFPSQMLRTGNNFTFSYTFEDVPFHSSYAHSQSLDRLMNPLIDQYLYYLSRTNTPSGTTTQSRLQFSQAGASDIRDQSRNWLPGPCYRQQRVSKTSADNNNSEYSWTGATKYHLNGRDSLVNPGPAMASHKDDEEKFFPQSGVLIFGKQGSEKTNVDIEKVMITDEEEIRTTNPVATEQYGSVSTNLQRGNLASNTTQKTARQAATADVNTQGVLPGMVWQDRDVYLQGPIWAKIPHTDGHFHPSPLMGGFGLKHPPPQILIKNTPVPANPSTTFSAAKFASFITQYSTGQVSVEIEWELQKENSKRWNPEIQYTSNYNKSVNVDFTVDTNGVYSEPRPIGTRYLTRNL

SEQ ID NO: 61 - protein, 745 aa, Artificial Sequence
  variant AAV capsid
MAADGYLPDWLEDTLSEGIRQWWKLKPGPPPPKPAERHKDDSRGLVLPGYKYLGPFNGLDKGEPVNEADAAALEHDKAYDRQLDSGDNPYLKYNHADAEFQERLKEDTSFGGNLGRAVFQAKKRVLEPLGLVEEPVKTAPGKKRPVEHSPVEPDSSSGTGKAGQQPARKRLNFGQTGDADSVPDPQPLGQPPAAPSGLGTNTMATGSGAPMADNNEGADGVGNSSGNWHCDSTWMGDRVITTSTRTWALPTYNNHLYKQISSQSGASNDNHYFGYSTPWGYFDFNRFHCHFSPRDWQRLINNNWGFRPKRLNFKLFNIQVKEVTQNDGTTTIANNLTSTVQVFTDSEYQLPYVLGSAHQGCLPPFPADVFMVPQYGYLTLNNGSQAVGRSSFYCLEYFPSQMLRTGNNFTFSYTFEDVPFHSSYAHSQSLDRLMNPLIDQYLYYLSRTNTPSGTTTQSRLQFSQAGASDIRDQSRNWLPGPCYRQQRVSKTSADNNNSEYSWTGATKYHLNGRDSLVNPGPAMASHKDDEEKFFPQSGVLIFGKQGSEKTNVDIEKVMITDEEEIRTTNPVATEQYGSVSTNLQRGNLAASDSTKAARQAATADVNTQGVLPGMVWQDRDVYLQGPIWAKIPHTDGHFHPSPLMGGFGLKHPPPQILIKNTPVPANPSTTFSAAKFASFITQYSTGQVSVEIEWELQKENSKRWNPEIQYTSNYNKSVNVDFTVDTNGVYSEPRPIGTRYLTRNL

SEQ ID NO: 62 - protein, 725 aa, Artificial Sequence
  Variant AAV capsid chimera
MAADGYLPDWLEDNLSEGIREWWDLKPGAPKPKANQQKQDDGRGLVLPGYKYLGPFNGLDKGEPVNAADAAALEHDKAYDQQLKAGDNPYLRYNHADAEFQERLQEDTSFGGNLGRAVFQAKKRVLEPFGLVEEGAKTAPTGKRIDDHFPKRKKARTEEDSKPSTSSDAEAGPSGSQQLQIPAQPASSLGADTMSAGGGGPLGDNNQGADGVGNASGDWHCDSTWMGDRIVTKSTRTWVLPSYNNHQYREIKSGSVDGSNANAYFGYSTPWGYFDFNRFHSHWSPRDWQRLINNYWGFRPRSLRVKIFNIQVKEVTVQDSTTTIANNLTSTVQVFTDDDYQLPYVVGNGTEGCLPAFPPQVFTLPQYGYATLNRDNTENPTERSSFFCLEYFPSKMLRTGNNFEFTYNFEEVPFHSSFAPSQNLFKLANPLVDQYLYRFVSTNNTGGVQFNKNLAGRYANTYKNWFPGPMGRTQGWNLGSGVNRASVSAFTTTNRMELEGASYQVPPQPNGMTNNLQGSNTYALENTMIFNSQPANPGTTATYLEGNMLITSESETQPVNRVAYNVGGQMATNNQSSTTAPTTGTYNLQEIVPGSVWMERDVYLQGPIWAKIPETGAHFHPSPAMGGFGLKHPPPMMLIKNTPVPGNITSFSDVPVSSFITQYSTGQVTVEMEWELKKENSKRWNPEIQYTNNYNDPQFVDFAPDSTGEYRTTRPIGTRYLTRPL

SEQ ID NO: 63 - protein, 725 aa, Artificial Sequence
  Variant AAV capsid chimera
MAADGYLPDWLEDTLSEGIRQWWKLKPGPPPPKPAERHKDDSRGLVLPGYKYLGPFNGLDKGEPVNAADAAALEHDKAYDQQLKAGDNPYLRYNHADAEFQERLQEDTSFGGNLGRAVFQAKKRVLEPFGLVEEGAKTAPTGKRIDDHFPKRKKARTEEDSKPSTSSDAEAGPSGSQQLQIPAQPASSLGADTMSAGGGGPLGDNNQGADGVGNASGDWHCDSTWMGDRIVTKSTRTWVLPSYNNHQYREIKSGSVDGSNANAYFGYSTPWGYFDFNRFHSHWSPRDWQRLINNYWGFRPRSLRVKIFNIQVKEVTVQDSTTTIANNLTSTVQVFTDDDYQLPYVVGNGTEGCLPAFPPQVFTLPQYGYATLNRDNTENPTERSSFFCLEYFPSKMLRTGNNFEFTYNFEEVPFHSSFAPSQNLFKLANPLVDQYLYRFVSTNNTGGVQFNKNLAGRYANTYKNWFPGPMGRTQGWNLGSGVNRASVSAFTTTNRMELEGASYQVPPQPNGMTNNLQGSNTYALENTMIFNSQPANPGTTATYLEGNMLITSESETQPVNRVAYNVGGQMATNNQSSTTAPTTGTYNLQEIVPGSVWMERDVYLQGPIWAKIPETGAHFHPSPAMGGFGLKHPPPMMLIKNTPVPGNITSFSDVPVSSFITQYSTGQVTVEMEWELKKENSKRWNPEIQYTNNYNDPQFVDFAPDSTGEYRTTRPIGTRYLTRPL

SEQ ID NO: 64 - protein, 3685 aa, Homo sapiens
MLWWEEVEDCYEREDVQKKTFTKWVNAQFSKFGKQHIENLFSDLQDGRRLLDLLEGLTGQKLPKEKGSTRVHALNNVNKALRVLQNNNVDLVNIGSTDIVDGNHKLTLGLIWNIILHWQVKNVMKNIMAGLQQTNSEKILLSWVRQSTRNYPQVNVINFTTSWSDGLALNALIHSHRPDLFDWNSVVCQQSATQRLEHAFNIARYQLGIEKLLDPEDVDTTYPDKKSILMYITSLFQVLPQQVSIEAIQEVEMLPRPPKVTKEEHFQLHHQMHYSQQITVSLAQGYERTSSPKPRFKSYAYTQAAYVTTSDPTRSPFPSQHLEAPEDKSFGSSLMESEVNLDRYQTALEEVLSWLLSAEDTLQAQGEISNDVEVVKDQFHTHEGYMMDLTAHQGRVGNILQLGSKLIGTGKLSEDEETEVQEQMNLLNSRWECLRVASMEKQSNLHRVLMDLQNQKLKELNDWLTKTEERTRKMEEEPLGPDLEDLKRQVQQHKVLQEDLEQEQVRVNSLTHMVVVVDESSGDHATAALEEQLKVLGDRWANICRWTEDRWVLLQDILLKWQRLTEEQCLFSAWLSEKEDAVNKIHTTGFKDQNEMLSSLQKLAVLKADLEKKKQSMGKLYSLKQDLLSTLKNKSVTQKTEAWLDNFARCWDNLVQKLEKSTAQISQAVTTTQPSLTQTTVMETVTTVTTREQILVKHAQEELPPPPPQKKRQITVDSEIRKRLDVDITELHSWITRSEAVLQSPEFAIFRKEGNFSDLKEKVNAIEREKAEKFRKLQDASRSAQALVEQMVNEGVNADSIKQASEQLNSRWIEFCQLLSERLNWLEYQNNIIAFYNQLQQLEQMTTTAENWLKIQPTTPSEPTAIKSQLKICKDEVNRLSGLQPQIERLKIQSIALKEKGQGPMFLDADFVAFTNHFKQVFSDVQAREKELQTIFDTLPPMRYQETMSAIRTWVQQSETKLSIPQLSVTDYEIMEQRLGELQALQSSLQEQQSGLYYLSTTVKEMSKKAPSEISRKYQSEFEEIEGRWKKLSSQLVEHCQKLEEQMNKLRKIQNHIQTLKKWMAEVDVFLKEEWPALGDSEILKKQLKQCRLLVSDIQTIQPSLNSVNEGGQKIKNEAEPEFASRLETELKELNTQWDHMCQQVYARKEALKGGLEKTVSLQKDLSEMHEWMTQAEEEYLERDFEYKTPDELQKAVEEMKRAKEEAQQKEAKVKLLTESVNSVIAQAPPVAQEALKKELETLTTNYQWLCTRLNGKCKTLEEVWACWHELLSYLEKANKWLNEVEFKLKTTENIPGGAEEISEVLDSLENLMRHSEDNPNQIRILAQTLTDGGVMDELINEELETFNSRWRELHEEAVRRQKLLEQSIQSAQETEKSLHLIQESLTFIDKQLAAYIADKVDAAQMPQEAQKIQSDLTSHEISLEEMKKHNQGKEAAQRVLSQIDVAQKKLQDVSMKFRLFQKPANFEQRLQESKMILDEVKMHLPALETKSVEQEVVQSQLNHCVNLYKSLSEVKSEVEMVIKTGRQIVQKKQTENPKELDERVTALKLHYNELGAKVTERKQQLEKCLKLSRKMRKEMNVLTEWLAATDMELTKRSAVEGMPSNLDSEVAWGKATQKEIEKQKVHLKSITEVGEALKTVLGKKETLVEDKLSLLNSNWIAVTSRAEEWLNLLLEYQKHMETFDQNVDHITKWIIQADTLLDESEKKKPQQKEDVLKRLKAELNDIRPKVDSTRDQAANLMANRGDHCRKLVEPQISELNHRFAAISHRIKTGKASIPLKELEQFNSDIQKLLEPLEAEIQQGVNLKEEDFNKDMNEDNEGTVKELLQRGDNLQQRITDERKREEIKIKQQLLQTKHNALKDLRSQRRKKALEISHQWYQYKRQADDLLKCLDDIEKKLASLPEPRDERKIKEIDRELQKKKEELNAVRRQAEGLSEDGAAMAVEPTQIQLSKRWREIESKFAQFRRLNFAQIHTVREETMMVMTEDMPLEISYVPSTYLTEITHVSQALLEVEQLLNAPDLCAKDFEDLFKQEESLKNIKDSLQQSSGRIDIIHSKKTAALQSATPVERVKLQEALSQLDFQWEKVNKMYKDRQGRFDRSVEKWRRFHYDIKIFNQWLTEAEQFLRKTQIPENWEHAKYKWYLKELQDGIGQRQTVVRTLNATGEEIIQQSSKTDASILQEKLGSLNLRWQEVCKQLSDRKKRLEEQKNILSEFQRDLNEFVLWLEEADNIASIPLEPGKEQQLKEKLEQVKLLVEELPLRQGILKQLNETGGPVLVSAPISPEEQDKLENKLKQTNLQWIKVSRALPEKQGEIEAQIKDLGQLEKKLEDLEEQLNHLLLWLSPIRNQLEIYNQPNQEGPFDVQETEIAVQAKQPDVEEILSKGQHLYKEKPATQPVKRKLEDLSSEWKAVNRLLQELRAKQPDLAPGLTTIGASPTQTVTLVTQPVVTKETAISKLEMPSSLMLEVPALADFNRAWTELTDWLSLLDQVIKSQRVMVGDLEDINEMIIKQKATMQDLEQRRPQLEELITAAQNLKNKTSNQEARTIITDRIERIQNQWDEVQEHLQNRRQQLNEMLKDSTQWLEAKEEAEQVLGQARAKLESWKEGPYTVDAIQKKITETKQLAKDLRQWQTNVDVANDLALKLLRDYSADDTRKVHMITENINASWRSIHKRVSEREAALEETHRLLQQFPLDLEKFLAWLTEAETTANVLQDATRKERLLEDSKGVKELMKQWQDLQGEIEAHTDVYHNLDENSQKILRSLEGSDDAVLLQRRLDNMNFKWSELRKKSLNIRSHLEASSDQWKRLHLSLQELLVWLQLKDDELSRQAPIGGDFPAVQKQNDVHRAFKRELKTKEPVIMSTLETVRIFLTEQPLEGLEKLYQEPRELPPEERAQNVTRLLRKQAEEVNTEWEKLNLHSADWQRKIDETLERLQELQEATDELDLKLRQAEVIKGSWQPVGDLLIDSLQDHLEKVKALRGEIAPLKENVSHVNDLARQLTTLGIQLSPYNLSTLEDLNTRWKLLQVAVEDRVRQLHEAHRDFGPASQHFLSTSVQGPWERAISPNKVPYYINHETQTTCWDHPKMTELYQSLADLNNVRFSAYRTAMKLRRLQKALCLDLLSLSAACDALDQHNLKQNDQPMDILQIINCLTTIYDRLEQEHNNLVNVPLCVDMCLNWLLNVYDTGRTGRIRVLSFKTGIISLCKAHLEDKYRYLFKQVASSTGFCDQRRLGLLLHDSIQIPRQLGEVASFGGSNIEPSVRSCFQFANNKPEIEAALFLDWMRLEPQSMVWLPVLHRVAAAETAKHQAKCNICKECPIIGFRYRSLKHFNYDICQSCFFSGRVAKGHKMHYPMVEYCTPTTSGEDVRDFAKVLKNKFRTKRYFAKHPRMGYLPVQTVLEGDNMETPVTLINFWPVDSAPASSPQLSHDDTHSRIEHYASRLAEMENSNGSYLNDSISPNESIDDEHLLIQHYCQSLNQDSPLSQPRSPAQILISLESEERGELERILADLEEENRNLQAEYDRLKQQHEHKGLSPLPSPPEMMPTSPQSPRDAELIAEAKLLRQHKGRLEARMQILEDHNKQLESQLHRLRQLLEQPQAEAKVNGTTVSSPSTSLQRSDSSQPMLLRVVGSQTSDSMGEEDLLSPPQDTSTGLEEVMEQLNNSFPSSRGRNTPGKPMREDTM

SEQ ID NO: 65 - DNA, 19841 bp, Homo sapiens
tttcctacttgaagcctgacgtagtaaagatcgggggagggttagacagatacagtggtccccaaccattttggcaccagggactggtcttatggaagacagtttttccacagactgttggggggatggttttgggatgaaaccgttctgcctctgatcatcaggtgttagattctaataaggagcgcacacctagatccctcgcatgcatagttcatggtggggttcgcactcttacgaggattgaatggtgcgctgctccggtaggaggctgggctcaggctgtaatgcctgctcgcccaccactcacctcctgctgcatggcctggttcctaacaggccacggaccactactgttccatggcccggaggttgaggaccccgagatacaggacaattctgtggcaagcaggactgtcccctcgccaaagatgggacatcgaggctccttggagcaccctgtggccaccttgcagcagcctctgtttccccatgtttccatgacctggtgtccatctgtcttccccagtttgggagcttctctccgaggaggacctgggcctggtgtggcacctgctgtgtgagcggggccatgtccaacggccttcttggggactttgggtcggggagaagttctgcctgggttttactgccttctcccaaccccacactgtctcccctggcagcggttgatcgacaagaccaaggtgacatatctgaagtggctgcctgagtcggagagcctgttcctggcatcacacgccagtggccacctgtacctgtacaacgtcagccacccctgcgcctcggccccgccccagtacagcctgctgaagcagggcgagggcttctctgtctatgctgccaagagcaaggcaccccgcaacccgctggccaagtgggcggtgggtgaggggcccctcaacgagttcgccttctcgcccgatggccggcacctggcctgtgtgagccaggatggctgcctgcgcgtcttccacttcgactccatgctcctgcgtgggctcatgaagagctactttgggggcctgctgtgtgtgtgctggagccctgacggccgctacgtggtgacgggtggcgaagatgacctggtcaccgtgtggtccttcaccgagggccgcgtggtggctcgaggccatggccacaagtcctgggtcaacgctgtggcctttgacccctacaccacaagggcagaggaggcggcgacagcagccggtgctgatggggagcggagcggcgaagaggaggaggaggagcccgaggctgcgggcacaggctcggccgggggcgccccgctctctccactgcccaaggctggctccattacttaccgctttggctcggcgggccaggacacgcagttctgcctgtgggacctcactgaagacgtgctctacccgcacccccccctggcccgcacccgcaccctccctggcacacctggcaccacgccaccggccgccagcagctcgaggggtggcgagcctggcccaggccccctgcctcgctcgctgtcccgctccaacagtctcccgcacccagctggcgggggcaaggcgggcggcccgggtgtggcggcagagcctggcacaccattcagcattggccgcttcgccacgctcacactgcaggagcggcgggaccggggggcagagaaggagcacaagcgctaccacagcctgggcaacatcagccggggtggcagtggcggcagtggcagtggtggggagaagcccagcggccctgttccccgcagccgcctggaccccgccaaggtgctgggcactgcgctgtgcccgcgcatccacgaggtgcccctgctggagccccttgtgtgcaagaagatcgcccaggagcggctcacagtcctcctgttcctggaggactgcatcatcactgcctgccaggagggcctcatctgcacctgggcccggccgggcaaggcggtgagtggccccacaccagcctgccggggacctggcaggacctttcgtgggaagaggcaggcattggcagagagagggctttgttgctgtcacagcctctggctccgtggggtgaggggaagccagggaaatcttagtgtctcagtacaagacctctcagatccttagagtgagggggtctagccctaggcagcaggcagcagaaagaggggtgggtgtgagagccagctaggaattggggcatccaaggctggccgtctgaagggcagcagatgggccccacatggccaggtcttactgcctgtcactcgaaccagaatctatttctgttgaacatctgttttttaaatcgtgaaacttttttgagtacttcaggccaaaactaggggcgagctcaagcctgtgggcatggctgccagcctgggtctgggactcaggatctgagcctcctgctgaaggcacaggctgggaatcccaggcctgggttccagtcccactccctctgtgaccctggacaagtcactgccccctctgacctccaactcatcacctcttagaacagagcctgtaggatgggcagtgggtggatgtgcttgcctcctgggtgggctgtggcgttgggaaggtcatagtaggcgaatcaggcctggcatcttgtaagttcggagctcgtcttgggtgtctcagcttcttagggcttggactcagttgcccagggtcctggaggccgtggcttggttcctcagatcctcagttttggaatcgtagagtcctgagtccctagaacttgagagcacagtctgagtgactcagaggcaagagtggtgggatttggggagtctggttgagtcctaaaagagacccctctgtctccgtagttcacagacgaggagaccgaggcccagacaggggaaggaagttggcccaggtcacccagcaagtcagtggtagaggtaggactgtccctgagttctttccccagcacctcagggtccctcccaagttagaagggagctccagtttccccctcccctcccacccttacccttaccccatggtctcactcaggatccgccaaggactttgattattgcgtgaaagtgctgactgccaggacaggaagctagctaagatgcaagttcccagcctagagcagtggcctctggggggtctagggcggacccaagggcaaggccagggtggcagcagctttggggactctgggctggctccctccccttgacactggctgaagcccaggtggtctctaacccctcccatctctccctctcatcttccccagggcatctcctcccaaccaggcaactccccgagtggcacagtggtgtgaagccatggatatcgggcccccccaaccccatgcccccagcctcctagccataaccctccctgctgacctcacagatcaacgtattaacaagactaaccatgatggatggactgctccagtccccccacctgcacaaaatttgggggccccccagactggcccggacacgggcgatgtaatagcccttgtggcctcagccttgtcccccacccactgccaagtacaatgacctcttcctctgaaacatcagtgttaccctcatccctgtccccagcatgtgactggtcactcctggggagagactccccgcccctgccacaagagccccaggtctgcagtgtgcccctcagttgagtgggcagggccgggggtggtccagccctcgcccggcccccaccccagctgcccttgctattgtctgtgcttttgaagagtgttaaattatggaagcccctcaggttcctccctgtcccgcaggacctcttatttatactaaagttccctgttttctcagcgggtctgtccccttcggaggagatgatgtagaggacctgtgtgtgtactctgtggttctaggcagtccgctttccccagaggaggagtgcaggcctgctcccagcccagcgcctcccaccccttttcatagcaggaaaagccggagcccagggagggaacggacctgcgagtcacacaactggtgacccacaccagcggctggagcaggaccctcttggggagaagagcatcctgcccgcagccagggcccctcatcaaagtcctcggtgttttttaaattatcagaactgcccaggaccacgtttcccaggccctgcccagctgggactcctcggtccttgcctcctagtttctcaggcctggccctctcaaggcccaggcaccccaggccggttggaggccccgacttccactctggagaaccgtccaccctggaaagaagagctcagattcctcttggctctcggagccgcagggagtgtgtcttcccgcgccaccctccaccccccgaaatgtttctgtttctaatcccagcctgggcaggaatgtggctccccggccaggggccaaggagctattttggggtctcgtttgcccagggagggcttggctccaccactttcctcccccagcctttgggcagcaggtcacccctgttcaggctctgagggtgccccctcctggtcctgtcctcaccaccccttccccacctcctgggaaaaaaaaaaaaaaaaaaaaaaaaagctggtataaagcagagagcctgagggctaaatttaactgtccgagtcggaatccatctctgagtcacccaagaagctgccctggcctcccgtccccttcccaggcctcaacccctttctcccacccagccccaacccccagccctcaccccctagcccccagttctggagcttgtcgggagcaagggggtggttgctactgggtcactcagcctcaattggccctgtttcagcaatgggcaggttcttcttgaaattcatcacacctgtggcttcctctgtgctctacctttttattggggtgacagtgtgacagctgagattctccatgcattccccctactctagcactgaagggttctgaagggccctggaaggagggagcttggggggctggcttgtgaggggttaaggctgggaggcgggaggggggctggaccaaggggtggggagaaggggaggaggcctcggccggccgcagagagaagtggccagagaggcccaggggacagccagggacaggcagacatgcagccagggctccagggcctggacaggggctgccaggccctgtgacaggaggaccccgagcccccggcccggggaggggccatggtgctgcctgtccaacatgtcagccgaggtgcggctgaggcggctccagcagctggtgttggacccgggcttcctggggctggagcccctgctcgaccttctcctgggcgtccaccaggagctgggcgcctccgaactggcccaggacaagtacgtggccgacttcttgcagtggggtgagtgcctaccctcggggctcctgcagatggggtgggggtggggcaggagacaggtctgggcacagaggcctggctgttgggggggcaggatggcaggatgggcatggggagatcctcccatcctggggctcagagtgtggacctgggccctggggcaacatttctctgtcctatgccaccactctggaggggcagagtaaggtcagcagaggctagggtggctgtgactcagagccatggcttaggagtcacagcaggctaggctgccaacagcctcccatggcctctctgcaccccgcctcagggtcagggtcagggtcatgctgggagctccctctcctaggaccctccccccaaaagtgggctctatggccctctcccctggtttcctgtggcctggggcaagccaggagggccagcatggggcagctgccaggggcgcagccgacaggcaggtgttcggcgccagcctctccagctgccccaacaggtgcccaggcactgggagggcggtgactcacgcgggccctgtgggagaaccagctttgcagacaggcgccaccagtgccccctcctctgcgatccaggagggacaactttgggttcttctgggtgtgtctccttcttttgtaggttctgcacccacccccacccccagccccaaagtctcggttcctatgagccgtgtgggtcagccaccattcccgccaccccgggtccctgcgtcctttagttctcctggcccagggcctccaaccttccagctgtcccacaaaaccccttcttgcaagggctttccagggcctggggccagggctggaaggaggatgcttccgcttctgccagctgccttgtctgcccacctcctccccaagcccaggactcgggctcactggtcactggtttctttcattcccagcaccctgcccctctggccctcatatgtctggccctcagtgactggtgtttggtttttggcctgtgtgtaacaaactgtgtgtgacacttgtttcctgtttctccgccttcccctgcttcctcttgtgtccatctctttctgacccaggcctggttcctttccctcctcctcccatttcacagatgggaaggtggaggccaagaagggccaggccattcagcctctggaaaaaccttctcccaacctcccacagcccctaatgactctcctggcctccctttagtagaggatgaagttgggttggcagggtaaactgagaccgggtggggtaggggtctggcgctcccgggaggagcactccttttgtggcccgagctgcatctcgcggcccctcccctgccaggcctggggcgggggagggggccagggttcctgctgccttaaaagggctcaatgtcttggctctctcctccctcccccgtcctcagccctggctggttcgtccctgctggcccactctcccggaaccccccggaacccctctctttcctccagaacccactgtctcctctccttccctcccctcccatacccatccctctctccatcctgcctccacttcttccacccccgggagtccaggcctccctgtccccacagtccctgagccacaagcctccaccccagctggtcccccacccaggctgcccagtttaacattcctagtcataggaccttgacttctgagaggcctgattgtcatctgtaaataaggggtaggactaaagcactcctcctggaggactgagagatgggctggaccggagcacttgagtctgggatatgtgaccatgctacctttgtctccctgtcctgttccttcccccagccccaaatccagggttttccaaagtgtggttcaagaaccacctgcatctgaatctagaggtactggatacaaccccacgtctgggccgttacccaggacattctacatgagaacgtgggggtggggccctggctgcacctgaactgtcacctggagtcagggtggaaggtggaagaactgggtcttatttccttctccccttgttctttagggtctgtccttctgcagactccgttaccccaccctaaccatcctgcacacccttggagccctctgggccaatgccctgtcccgcaaagggcttctcaggcatctcacctctatgggagggcatttttggcccccagaaccttacacggtgtttatgtggggaagcccctgggaagcagacagtcctagggtgaagctgagaggcagagagaaggggagacagacagagggtggggctttcccccttgtctccagtgccctttctggtgaccctcggttcttttcccccaccacccccccagcggagcccatcgtggtgaggcttaaggaggtccgactgcagagggacgacttcgagattctgaaggtgatcggacgcggggcgttcagcgaggtaagccgaaccgggcgggagcctgacttgactcgtggtgggcggggcataggggttggggcggggccttagaaattgatgaatgaccgagccttagaacctagggctgggctggaggcggggcttgggaccaatgggcgtggtgtggcaggtggggcggggccacggctgggtgcagaagcgggtggagttgggtctgggcgagcccttttgttttcccgccgtctccactctgtctcactatctcgacctcaggtagcggtagtgaagatgaagcagacgggccaggtgtatgccatgaagatcatgaacaagtgggacatgctgaagaggggcgaggtgaggggctgggcggacgtggggggctttgaggatccgcgccccgtctccggctgcagctcctccgggtgccctgcaggtgtcgtgcttccgtgaggagagggacgtgttggtgaatggggaccggcggtggatcacgcagctgcacttcgccttccaggatgagaactacctggtgagctccgggccggggtgactaggaagagggacaagagcccgtgctgtcactggacgaggaggtggggagaggaagctctaggattgggggtgctgcccggaaacgtctgtgggaaagtctgtgtgcggtaagagggtgtgtcaggtggatgaggggccttccctatctgagacggggatggtgtccttcactgcccgtttctggggtgatctgggggactcttataaagatgtctctgttgcggggggtctcttacctggaatgggataggtcttcaggaattctaacggggccactgcctagggaaggagtgtctgggacctattctctgggtgttgggtggcctctgggttctctttcccagaacatctcagggggagtgaatctgcccagtgacatcccaggaaagtttttttgtttgtgtttttttttgaggggcgggggcgggggccgcaggtggtctctgatttggcccggcagatctctatggttatctctgggctggggctgcaggtctctgcccaaggatggggtgtctctgggaggggttgtcccagccatccgtgatggatcagggcctcaggggactaccaaccacccatgacgaaccccttctcagtacctggtcatggagtattacgtgggcggggacctgctgacactgctgagcaagtttggggagcggattccggccgagatggcgcgcttctacctggcggagattgtcatggccatagactcggtgcaccggcttggctacgtgcacaggtgggtgcagcatggccgaggggatagcaagcttgttccctggccgggttcttggaaggtcagagcccagagaggccagggcctggagagggaccttcttggttggggcccaccggggggtgcctgggagtaggggtcagaactgtagaagccctacaggggcggaacccgaggaagtggggtcccaggtggcactgcccggaggggcggagcctggtgggaccacagaagggaggttcatttatcccacccttctcttttcctccgtgcagggacatcaaacccgacaacatcctgctggaccgctgtggccacatccgcctggccgacttcggctcttgcctcaagctgcgggcagatggaacggtgagccagtgccctggccacagagcaactggggctgctgatgagggatggaaggcacagagtgtgggagcgggactggatttggaggggaaaagaggtggtgtgacccaggcttaagtgtgcatctgtgtggcggagtattagaccaggcagagggaggggctaagcatttggggagtggttggaaggagggcccagagctggtgggcccagaggggtgggcccaagcctcgctctgctccttttggtccaggtgcggtcgctggtggctgtgggcaccccagactacctgtcccccgagatcctgcaggctgtgggcggtgggcctgggacaggcagctacgggcccgagtgtgactggtgggcgctgggtgtattcgcctatgaaatgttctatgggcagacgcccttctacgcggattccacggcggagacctatggcaagatcgtccactacaaggtgagcacggccgcagggagacctggcctctcccggtaggcgctcccaggctatcgcctcctctccctctgagcaggagcacctctctctgccgctggtggacgaaggggtccctgaggaggctcgagacttcattcagcggttgctgtgtcccccggagacacggctgggccggggtggagcaggcgacttccggacacatcccttcttctttggcctcgactgggatggtctccgggacagcgtgcccccctttacaccggatttcgaaggtgccaccgacacatgcaacttcgacttggtggaggacgggctcactgccatggtgagcgggggcggggtaggtacctgtggcccctgctcggctgcgggaacctccccatgctccctccataaagttggagtaaggacagtgcctaccttctggggtcctgaatcactcattccccagagcacctgctctgtgcccatctactactgaggacccagcagtgacctagacttacagtccagtgggggaacacagagcagtcttcagacagtaaggccccagagtgatcagggctgagacaatggagtgcagggggtgggggactcctgactcagcaaggaaggtcctggagggctttctggagtggggagctatctgagctgagacttggagggatgagaagcaggagaggactcctcctcccttaggccgtctctcttcaccgtgtaacaagctgtcatggcatgcttgctcggctctgggtgcccttttgctgaacaatactggggatccagcacggaccagatgagctctggtccctgccctcatccagttgcagtctagagaattagagaattatggagagtgtggcaggtgccctgaagggaagcaacaggatacaagaaaaaatgatggggccaggcacggtggctcacgcctgtaaccccagcaatttggcaggccgaagtgggtggattgcttgagcccaggagttcgagaccagcctgggcaatgtggtgagacccccgtctctacaaaaatgttttaaaaattggttgggcgtggtggcgcatgcctgtatactcagctactagggtggccgacgtgggcttgagcccaggaggtcaaggctgcagtgagctgtgattgtgccactgcactccagcctgggcaacggagagagactctgtctcaaaaataagataaactgaaattaaaaaataggctgggctggccgggcgtggtggctcacgcctgtaatctcagcactttgggaggccgaggcgggtggatcacgaggtcaggagatcgagaccatcttggctaacacggtgaaaccccatctctcctaaaaatacaaaaaattagccaggcgtggtggcgggcgcctgtagtcccagctactcaggaggctgaggcaggagaatggcgtgaacccgggaggcagagtttgcagtgagccgagatcgtgccactgcactccagcctgggcgacagagcgagactctgtctcagaaaaaaaaaaaaaaaaaaaaaaaaataggctggaccgcggccgggcgctgtggctcatgcctgtaatcccagcactttgggagtccaaggccggtgggtcatgagatcaggagttttgagactaggctggccaacacggtgaaaccccgtctctactaaaaatacaagaaaattagctgggtgtggtctcgggtgcctgtaattccagttactggggaagctgaggcaggagaattgcttgaacctgggaggcagagtttgcagtgagccaagatcatgccactacactccagtctgggtgacagagtgagactctgtctcaaaaaaaaaaaaaaaaaaaagggttgggcaaggtggttcacgcctgtaatcccagaactttgggaggctgaggcaggcagatcactggaagtcaggagttcaagaccagcctggccaacatggtgaaaccctgtgtctactaaaaatacaaaatttagccaggcttggtggcgtatgcctgtaatgccagctactcaggaggctgaggcaggagaatcgcttgattgaacctgggaggcagagtttgcagtgggctggggttgtgccactgcactctaggctgggagacagcaagactccatctaaaaaaaaaaaacagaactgggctgggcacagtggcttatatttgtaatcccagcactttgggaggctgaggttggaggactgcttgagcccagagtttgggactacaacagctgaggtaggcggatcacttgaggtcagaagatggagaccagcctggccagcgtggcgaaaccccgtctctaccaaaaatataaaaaattagccaggcgtggtagagggcgcctgtaatctcagctactcaggacgctgaggcaggagaatcgcctgaacctgggaggcggaggttgcagtgagctgagattgcaccactgcactccagcctgggtaacagagcgagactccgtatcaaagaaaaagaaaaaagaaaaaatgctggaggggccactttagataagccctgagttggggctggtttggggggaacatgtaagccaagatcaaaaagcagtgaggggcccgccctgacgactgctgctcacatctgtgtgtcttgcgcaggagacactgtcggacattcgggaaggtgcgccgctaggggtccacctgccttttgtgggctactcctactcctgcatggccctcaggtaagcactgccctggacggcctccaggggccacgaggctgcttgagcttcctgggtcctgctccttggcagccaatggagttgcaggatcagtcttggaaccttactgttttgggcccaaagactcctaagaggccagagttggaggaccttaaattttcagatctatgtacttcaaaatgttagattgaattttaaaacctcagagtcacagactgggcttcccagaatcttgtaaccattaacttttacgtctgtagtacacagagccacaggacttcagaacttggaaaatatgaagtttagacttttacaatcagttgtaaaagaatgcaaattctttgaatcagccatataacaataaggccatttaaaagtattaatttaggcgggccgcggtggctcacgcctgtaatcctagcactttgggaggccaaggcaggtggatcatgaggtcaggagatcgagaccatcctggctaacacggtgaaaccccgtctctactaaaaatacaaaaaaattagccgggcatggtggcgggcgcttgcggtcccagctacttgggaggcgaggcaggagaatggcatgaacccgggaggcggagcttgcagtgagccgagatcatgccactgcactccagcctgggcgacagagcaagactccgtctcaaaaaaaaaaaaaaaaaagtatttatttaggccgggtgtggtggctcacgcctgtaattccagtgctttgggaggatgaggtgggtggatcacctgaggtcaggagttcgagaccagcctgaccaacgtggagaaacctcatctctactaaaaaacaaaattagccaggcgtggtggcatatacctgtaatcccagctactcaggaggctgaggcaggagaatcagaacccaggagggggaggttgtggtgagctgagatcgtgccattgcattccagcctgggcaacaagagtgaaacttcatctcaaaaaaaaaaaaaaaaaagtactaatttacaggctgggcatggtggctcacgcttggaatcccagcactttgggaggctgaagtggacggattgcttcagcccaggagttcaagaccagcctgagcaacataatgagaccctgtctctacaaaaaattgaaaaaatcgtgccaggcatggtggtctgtgcctgcagtcctagctactcaggagtctgaagtaggagaatcacttgagcctggagtttgaggcttcagtgagccatgatagattccagcctaggcaacaaagtgagacctggtctcaacaaaagtattaattacacaaataatgcattgcttatcacaagtaaattagaaaatacagataaggaaaaggaagttgatatctcgtgagctcaccagatggcagtggtccctggctcacacgtgtactgacacatgtttaaatagtggagaacaggtgtttttttggtttgtttttttccccttcctcatgctactttgtctaagagaacagttggttttctagtcagcttttattactggacaacattacacatactataccttatcattaatgaactccagcttgattctgaaccgctgcggggcctgaacggtgggtcaggattgaacccatcctctattagaacccaggcgcatgtccaggatagctaggtcctgagccgtgttcccacaggagggactgctgggttggaggggacagccacttcataccccagggaggagctgtccccttcccacagctgagtggggtgtgctgacctcaagttgccatcttggggtcccatgcccagtcttaggaccacatctgtggaggtggccagagccaagcagtctccccatcaggtcggcctccctgtcctgaggccctgagaagaggggtctgcagcggtcacatgtcaagggaggagatgagctgaccctagaacatgggggtctggaccccaagtccctgcagaaggtttagaaagagcagctcccaggggcccaaggccaggagaggggcagggcttttcctaagcagaggaggggctattggcctacctgggactctgttctcttcgctctgctgctccccttcctcaaatcaggaggtcttggaagcagctgcccctacccacaggccagaagttctggttctccaccagagaatcagcattctgtctccctccccactccctcctcctctccccagggacagtgaggtcccaggccccacacccatggaactggaggccgagcagctgcttgagccacacgtgcaagcgcccagcctggagccctcggtgtccccacaggatgaaacagtaagttggtggaggggagggggtccgtcagggacaattgggagagaaaaggtgagggcttcccgggtggcgtgcactgtagagccctctagggacttcctgaacagaagcagacagaaaccacggagagacgaggttacttcagacatgggacggtctctgtagttacagtggggcattaagtaagggtgtgtgtgttgctggggatctgagaagtcgatctttgagctgagcgctggtgaaggagaaacaagccatggaaggaaaggtgccaagtggtcaggcgagagcctccagggcaaaggccttgggcaggtgggaatcctgatttgttcctgaaaggtagtttggctgaatcattcctgagaaggctggagaggccagcaggaaacaaaacccagcaaggccttttgtcgtgagggcattagggagctggagggattttgagcagcagagggacataggttgtgttagtgtttgagcaccagccctctggtccctgtgtagatttagaggaccagactcagggatggggctgagggaggtagggaagggagggggcttggatcattgcaggagctatggggattccagaaatgttgaggggacggaggagtaggggataaacaaggattcctagcctggaaccagtgcccaagtcctgagtcttccaggagccacaggcagccttaagcctggtccccatacacaggctgaagtggcagttccagcggctgtccctgcggcagaggctgaggccgaggtgacgctgcgggagctccaggaagccctggaggaggaggtgctcacccggcagagcctgagccgggagatggaggccatccgcacggacaaccagaacttcgccaggtcgggatcggggccggggccggggccgggatgcgggccggtggcaacccttggcatcccctctcgtccggcccggacggactcaccgtccttacctccccacagtcaactacgcgaggcagaggctcggaaccgggacctagaggcacacgtccggcagttgcaggagcggatggagttgctgcaggcagagggagccacaggtgagtccctcatgtgtccccttccccggaggaccgggaggaggtgggccgtctgctccgcggggcgtgtatagacacctggaggagggaagggacccacgctggggcacgccgcgccaccgccctccttcgcccctccacgcgccctatgcctctttcttctccttccagctgtcacgggggtccccagtccccgggccacggatccaccttcccatgtaagacccctctctttcccctgcctcagacctgctgcccattctgcagatcccctccctggctcctggtctccccgtccagatatagggctcaccctacgtctttgcgactttagagggcagaagccctttattcagccccagatctccctccgttcaggcctcaccagattccctccgggatctccctagataacctccccaacctcgattcccctcgctgtctctcgccccaccgctgagggctgggctgggctccgatcgggtcacctgtcccttctctctccagctagatggccccccggccgtggctgtgggccagtgcccgctggtggggccaggccccatgcaccgccgccacctgctgctccctgccagggtacgtccggctgcccacgcccccctccgccgtcgcgccccgcgctccacccgccccttgccacccgcttagctgcgcatttgcggggctgggcccacggcaggagggcggatcttcgggcagccaatcaacacaggccgctaggaagcagccaatgacgagttcggacgggattcgaggcgtgcgagtggactaacaacagctgtaggctgttggggcgggggcggggcgcagggaagagtgcgggcccacctatgggcgtaggcggggcgagtcccaggagccaatcagaggcccatgccgggtgttgacctcgccctctccccgcaggtccctaggcctggcctatcggaggcgctttccctgctcctgttcgccgttgttctgtctcgtgccgccgccctgggctgcattgggttggtggcccacgccggccaactcaccgcagtctggcgccgcccaggagccgcccgcgctccctgaaccctagaactgtcttcgactccggggccccgttggaagactgagtgcccggggcacggcacagaagccgcgcccaccgcctgccagttcacaaccgctccgagcgtgggtctccgcccagctccagtcctgtgatccgggcccgccccctagcggccggggagggaggggccgggtccgcggccggcgaacggggctcgaagggtccttgtagccgggaatgctgctgctgctgctgctgctgctgctgctgctgctgctgctgctgctgctgctgctgctggggggatcacagaccatttctttctttcggccaggctgaggccctgacgtggatgggcaaactgcaggcctgggaaggcagcaagccgggccgtccgtgttccatcctccacgcacccccacctatcgttggttcgcaaagtgcaaagctttcttgtgcatgacgccctgctctggggagcgtctggcgcgatctctgcctgcttactcgggaaatttgcttttgccaaacccgctttttcggggatcccgcgcccccctcctcacttgcgctgctctcggagccccagccggctccgcccgcttcggcggtttggatatttattgacctcgtcctccgactcgctgacaggctacaggacccccaacaaccccaatccacgttttggatgcactgagaccccgacattcctcggtatttattgtctgtccccacctaggacccccacccccgaccctcgcgaataaaaggccctccatctgcccaaagctctggactccacagtgtccgcggtttgcgttgtgggccggaggctccgcagcgggccaatccggaggcgtgtggaggcggccgaaggtctgggaggagctagcgggatgcgaagcggccgaatcagggttgggggaggaaaagccacggggcggggctttggcgtccggccaataggagggcgagcgggccacccggaggcaccgcccccgcccagctgtggcccagctgtgccaccgagcgtcgagaagagggggctgggctggcagcgcgcgcggccatcctccttccactgcgcctgcgcacgccacgcgcatccgctcctgggacgcaagctcgagaaaagttgctgcaaactttctagcccgttccccgcccctcctcccggccagacccgccccccctgcggagccgggaattccgaggggcggagcgcaggccgagatggggaatgtgggggcctgcagaggaccctggagacggaggcgtgcagaagctcagtctcggggcggaggcttcgcgcccttagtcctcctggacggcccgttaccttctgcgttgtcccgatggggaaactgaggccctgagccagaagcacacgctggggggaggcagaaagcgcggccagaggcggagggaaaacaaagggagaatcacagacagacgggagggggacggacacacacaaggggacagagacccgagtggagagctggatctcgccttcccggcgtggggcgcagggtcggccagaaagaagatcgagaagagcggggagtgggggcgaaaaggggggacaggtgggggaggaggctggggaaagcccgagggaggaagagagggagggaggaacttcccaaagttgcaaaacatggctaccttgcctgcggagccgagcgcggggccggcggctgggggggaggcggtggcggcggcggcggcgaccgaagaggaggaggaggaagcgcgccagctcttgcagactttgcaggcggccgagggtgaggcggcggcggcggccggggccggggcgggcgcagcggctgcgggagctgagggcccgggatccccgggcgtccccgggtcgccccccgaggccgcttccgaaccgcccacgggcctccgcttctcgcccgagcaggtggcgtgcgtctgcgaggcgctgctccaggcgggccacgccggccgcttgagccgcttcctgggcgcactgcccccggccgagcgcctacgtggcagcgacccggtgttgcgcgcgcgggccctggtggccttccagcggggcgagtacgccgagctctaccggctactcgagagccgccccttccccgccgcccaccacgccttcctgcaggacctctacctgcgcgcgcgctaccatgaggccgagcgggcccgcggccgcgcgcttggcgcagtggacaagtatcgactgcgcaagaagttcccgctgcccaagaccatctgggacggcgaggagacagtctactgcttcaaggagcgctcccgcgcagcgctcaaggcctgctaccgcggcaaccgctaccccacgccggacgagaagcgccgcctggccacactcaccggcctgtcgctcacgcaggtcagcaactggttcaagaaccggcgacagcgcgaccggaccggggccggaggcggcgcgccctgcaagaggtgaggggcctcgggcggcgcaagtccagctctcccggggacatcccgtccaccagccctcttcccccgtgcccactgctggggccggcgcgccgaggtcctcggacatctcccgggaccagctcacaatctcaggcgcccgcggggcgcggggactaagtgtggacgggacaggcacccgcccgggccctctccccgcacgcgtctcctcttccagcggctccattccgagctccttcccaaatcccatcggtgttggggaatcacactgcggggggcactagagggactgaggaaaaaggacagggcctgtggccactccact

SEQ ID NO: 66 - protein, 842 aa, Homo sapiens
MSRPLSDQEKRKQISVRGLAGVENVTELKKNFNRHLHFTLVKDRNVATPRDYYFALAHTVRDHLVGRWIRTQQHYYEKDPKRIYYLSLEFYMGRTLQNTMVNLALENACDEATYQLGLDMEELEEIEEDAGLGNGGLGRLAACFLDSMATLGLAAYGYGIRYEFGIFNQKISGGWQMEEADDWLRYGNPWEKARPEFTLPVHFYGHVEHTSQGAKWVDTQVVLAMPYDTPVPGYRNNVVNTMRLWSAKAPNDFNLKDFNVGGYIQAVLDRNLAENISRVLYPNDNFFEGKELRLKQEYFVVAATLQDIIRRFKSSKFGCRDPVRTNFDAFPDKVAIQLNDTHPSLAIPELMRILVDLERMDWDKAWDVTVRTCAYTNHTVLPEALERWPVHLLETLLPRHLQIIYEINQRFLNRVAAAFPGDVDRLRRMSLVEEGAVKRINMAHLCIAGSHAVNGVARIHSEILKKTIFKDFYELEPHKFQNKTNGITPRRWLVLCNPGLAEVIAERIGEDFISDLDQLRKLLSFVDDEAFIRDVAKVKQENKLKFAAYLEREYKVHINPNSLFDIQVKRIHEYKRQLLNCLHVITLYNRIKREPNKFFVPRTVMIGGKAAPGYHMAKMIIRLVTAIGDVVNHDPAVGDRLRVIFLENYRVSLAEKVIPAADLSEQISTAGTEASGTGNMKFMLNGALTIGTMDGANVEMAEEAGEENFFIFGMRVEDVDKLDQRGYNAQEYYDRIPELRQVIEQLSSGFFSPKQPDLFKDIVNMLMHHDRFKVFADYEDYIKCQEKVSALYKNPREWTRMVIRNIATSGKFSSDRTIAQYAREIWGVEPSRQRLPAPDEAI

SEQ ID NO: 67 - protein, 429 aa, Homo sapiens
MQLRNPELHLGCALALRFLALVSWDIPGARALDNGLARTPTMGWLHWERFMCNLDCQEEPDSCISEKLFMEMAELMVSEGWKDAGYEYLCIDDCWMAPQRDSEGRLQADPQRFPHGIRQLANYVHSKGLKLGIYADVGNKTCAGFPGSFGYYDIDAQTFADWGVDLLKFDGCYCDSLENLADGYKHMSLALNRTGRSIVYSCEWPLYMWPFQKPNYTEIRQYCNHWRNFADIDDSWKSIKSILDWTSFNQERIVDVAGPGGWNDPDMLVIGNFGLSWNQQVTQMALWAIMAAPLFMSNDLRHISPQAKALLQDKDVIAINQDPLGKQGYQLRQGDNFEVWERPLSGLAWAVAMINRQEIGGPRSYTIAVASLGKGVACNPACFITQLLPVKRKLGFYEWTSRLRSHINPTGTVLLQLENTMQMSLKDLL

SEQ ID NO: 68 - protein, 952 aa, Homo sapiens
MGVRHPPCSHRLLAVCALVSLATAALLGHILLHDFLLVPRELSGSSPVLEETHPAHQQGASRPGPRDAQAHPGRPRAVPTQCDVPPNSRFDCAPDKAITQEQCEARGCCYIPAKQGLQGAQMGQPWCFFPPSYPSYKLENLSSSEMGYTATLTRTTPTFFPKDILTLRLDVMMETENRLHFTIKDPANRRYEVPLETPHVHSRAPSPLYSVEFSEEPFGVIVRRQLDGRVLLNTTVAPLFFADQFLQLSTSLPSQYITGLAEHLSPLMLSTSWTRITLWNRDLAPTPGANLYGSHPFYLALEDGGSAHGVFLLNSNAMDVVLQPSPALSWRSTGGILDVYIFLGPEPKSVVQQYLDVVGYPFMPPYWGLGFHLCRWGYSSTAITRQVVENMTRAHFPLDVQWNDLDYMDSRRDFTFNKDGFRDFPAMVQELHQGGRRYMMIVDPAISSSGPAGSYRPYDEGLRRGVFITNETGQPLIGKVWPGSTAFPDFTNPTALAWWEDMVAEFHDQVPFDGMWIDMNEPSNFIRGSEDGCPNNELENPPYVPGVVGGTLQAATICASSHQFLSTHYNLHNLYGLTEAIASHRALVKARGTRPFVISRSTFAGHGRYAGHWTGDVWSSWEQLASSVPEILQFNLLGVPLVGADVCGFLGNTSEELCVRWTQLGAFYPFMRNHNSLLSLPQEPYSFSEPAQQAMRKALTLRYALLPHLYTLFHQAHVAGETVARPLFLEFPKDSSTWTVDHQLLWGEALLITPVLQAGKAEVTGYFPLGTWYDLQTVPVEALGSLPPPPAAPREPAIHSEGQWVTLPAPLDTINVHLRAGYIIPLQGPGLTTTESRQQPMALAVALTKGGEARGELFWDDGESLEVLERGAYTQVIFLARNNTIVNELVRVTSEGAGLQLQKVTVLGVATAPQQVLSNGVPVSNFTYSPDTKVLDICVSLLMGEQFLVSWC

SEQ ID NO: 69 - protein, 210 aa, Homo sapiens
MWTLGRRAVAGLLASPSPAQAQTLTRVPRPAELAPLCGRRGLRTDIDATCTPRRASSNQRGLNQIWNVKKQSVYLMNLRKSGTLGHPGSLDETTYERLAEETLDSLAEFFEDLADKPYTFEDYDVSFGSGVLTVKLGGDLGTYVINKQTPNKQIWLSSPSSGPKRYDWTGKNWVYSHDGVSLHELLAAELTKALKTKLDLSSLAYSGKDA